European Patent Application EP 4 148 134 A1, published March 15, 2023. Title: CHIMERIC POLYPEPTIDES HAVING TARGETED BINDING SPECIFICITY. Applicant: THE SCRIPPS RESEARCH INSTITUTE BARBAS, Carlos F. III MERCER, Andrew LAMB, Brian M. GAJ, Thomas. The sequence listing filed with the application follows.

SEQUENCE LISTING (369 sequences)

SEQ ID NO: 1 - DNA, 864 bp, Artificial Sequence
  Synthetic construct
atggatcccattcgttcgcgcacgccaagtcctgcccgcgagcttctgcccggaccccaaccggatagggttcagccgactgcagatcgggggggggctccgcctgctggcggccccctggatggcttgcccgctcggcggacgatgtcccggacccggctgccatctccccctgcgccctcgcctgcgttctcggcgggcagcttcagcgatctgctccgtcagttcgatccgtcgcttcttgatacatcgcttcttgattcgatgcctgccgtcggcacgccgcatacagcggctgccccagcagagtgcgatgaggtgcaatcgggtctgcgtgcagccgatgacccgccacccaccgtgcgtgtcgctgtcactgcggcgcggccgccgcgcgccaagccggccccgcgacggcgtgcggcgcaaccctccgacgcttcgccggccgcgcaggtggatctacgcacgctcggctacagtcagcagcagcaagagaagatcaaaccgaaggtgcgttcgacagtggcgcagcaccacgaggcactggtgggccatgggtttacacacgcgcacatcgttgcgctcagccaacacccggcagcgttagggaccgttgctgtcacgtatcaggacataatcagggcgttgccagaggcgacacacgaagacatcgttggcgtcggcaaacagtggtccggcgcacgcgctctggaggccttgctcacggaggcgggggagttgagaggtccgccgttacagttggacacaggccaacttctcaagattgcaaaacgtggcggcgtgaccgcagtggaggcagtgcatgcatggcgcaatgcactgacgggtgcccccctgaac

SEQ ID NO: 2 - protein, 288 aa, Artificial Sequence
  Synthetic construct
MDPIRSRTPSPARELLPGPQPDRVQPTADRGGAPPAGGPLDGLPARRTMSRTRLPSPPAPSPAFSAGSFSDLLRQFDPSLLDTSLLDSMPAVGTPHTAAAPAECDEVQSGLRAADDPPPTVRVAVTAARPPRAKPAPRRRAAQPSDASPAAQVDLRTLGYSQQQQEKIKPKVRSTVAQHHEALVGHGFTHAHIVALSQHPAALGTVAVTYQDIIRALPEATHEDIVGVGKQWSGARALEALLTEAGELRGPPLQLDTGQLLKIAKRGGVTAVEAVHAWRNALTGAPLN

SEQ ID NO: 3 - protein, 11 aa, Artificial Sequence
  Synthetic construct
  MISC_FEATURE (4)..(4): Xaa is Y, S or R
  MISC_FEATURE (5)..(5): Xaa is R or G
  MISC_FEATURE (6)..(6): Xaa is R, H, A, N or T
VGKXXXGARAL

SEQ ID NO: 4 - protein, 10 aa, Artificial Sequence
  Synthetic construct
VGKYRGARAL

SEQ ID NO: 5 - protein, 11 aa, Artificial Sequence
  Synthetic construct
VGKSRSGARAL

SEQ ID NO: 6 - protein, 10 aa, Artificial Sequence
  Synthetic construct
VGKYHGARAL

SEQ ID NO: 7 - protein, 11 aa, Artificial Sequence
  Synthetic construct
VGKRGAGARAL

SEQ ID NO: 8 - protein, 13 aa, Artificial Sequence
  Synthetic construct
  MISC_FEATURE (7)..(7): Xaa is Y, S or R
  MISC_FEATURE (8)..(8): Xaa is W or G
  MISC_FEATURE (9)..(9): Xaa is R, H, A, N or T
IVDIAKXXXGDLA

SEQ ID NO: 9 - protein, 13 aa, Artificial Sequence
  Synthetic construct
IVDIARQWSGDLA

SEQ ID NO: 10 - protein, 12 aa, Artificial Sequence
  Synthetic construct
IVDIARYRGDLA

SEQ ID NO: 11 - protein, 13 aa, Artificial Sequence
  Synthetic construct
IVDIARSRSGDLA

SEQ ID NO: 12 - protein, 12 aa, Artificial Sequence
  Synthetic construct
IVDIARYHGDLA

SEQ ID NO: 13 - protein, 13 aa, Artificial Sequence
  Synthetic construct
IVDIARRGAGDLA

SEQ ID NO: 14 - protein, 9 aa, Artificial Sequence
  Synthetic construct
  misc_feature (4)..(6): Xaa can be any naturally occurring amino acid
VGKXXXGAR

SEQ ID NO: 15 - protein, 12 aa, Artificial Sequence
  Synthetic construct
  misc_feature (5)..(8): Xaa can be any naturally occurring amino acid
VDIAXXXXGDLA

SEQ ID NO: 16 - protein, 48 aa, Artificial Sequence
  Synthetic construct
NIHGNININSHDNNHDHDHDNSNNHDHDNSNSNNNNNINGNNNINNSN

SEQ ID NO: 17 - DNA, 26 bp, Artificial Sequence
  Synthetic construct
ataaaccccctccaaccaggtgctaa

SEQ ID NO: 18 - protein, 52 aa, Artificial Sequence
  Synthetic construct
NINGNININIHDHDHDHDHDNGHDHDNINIHDHDNINNNNNGNNHDNGNINI

SEQ ID NO: 19 - protein, 1446 aa, Artificial Sequence
  Synthetic construct
MDPIRSRTPSPARELLPGPQPDRVQPTADRGGAPPAGGPLDGLPARRTMSRTRLPSPPAPSPAFSAGSFSDLLRQFDPSLLDTSLLDSMPAVGTPHTAAAPAECDEVQSGLRAADDPPPTVRVAVTAARPPRAKPAPRRRAAQPSDASPAAQVDLRTLGYSQQQQEKIKPKVRSTVAQHHEALVGHGFTHAHIVALSQHPAALGTVAVTYQDIIRALPEATHEDIVGVGKQWSGARALEALLTEAGELRGPPLQLDTGQLLKIAKRGGVTAVEAVHAWRNALTGAPLNLTPDQVVAIASNIGGKQALETVQRLLPVLCQDHGLTPDQVVAIASHGGGKQALETVQRLLPVLCQDHGLTPDQVVAIASNIGGKQALETVQRLLPVLCQAHGLTPDQVVAIASNIGGKQALETVQRLLPVLCQDHGLTPAQVVAIASNSGGKQALETVQRLLPVLCQDHGLTPDQVVAIASHDGGKQALETLQRLLPVLCQDHGLTPDQVVAIANNNGGKQALETLQRLLPVLCQDHGLTPDQVVAIASHDGGKQALETVQRLLPVLCQDHGLTPDQVVAIASHDGGKQALETVQRLLPVLCQDHGLTPAQVVAIASHDGGKQALETVQRLLPVLCQDHGLTPDQVVAIASNSGGKQALETVQRLLPVLCQDHGLTPDQVVAIASNGGKQALETVQRLLPVLCQDHGLTPDQVVAIASNGGKQALETVQRLLPVQRLLPVLCQDHGLTQDQVVAIASHDGGKQALETVQRLLPVLCQDHGLTPDQVVAIASHDGGKQALETVQRLLPVLCQDHGLTPDQVVAIASNSGGKQALETVQRLLPVLCQDHGLTPDQVVAIASNSGGKQALETVQRLLPVLCQDHGLTPDQVVAIASNNGGKQALETVQRLLPVLCQDHGLTPDQVVAIANNNGGKQALETVQRLLPVLCQDHGLTPAQVVAIASNIGGKQALETVQRLLPVLCQDHGLTLDQVVAIASNGGSKQALETVQRLLPVLCQDHGLTPDQVVAIANNNGGKQALETVQRLLPVLCQDHGLTPDQVVAIASNIGGKQALETVQRLLPVLCQDHGLTLDQVVAIASNGGKQALETVQRLLPVLCQDHGLTPNQVVAIASNSGGKQALETVQRLLPVLCQDHGLTPNQVVAIASNGGKQALESIVAQLSRPDPALAALTNDHLVALACLGGRPALDAVKKGLPHAPELIRRINRRIPERTSHRVPDLAHVVRVLGFFQSHSHPAQAFDDAMTQFEMSRHGLVQLFRRVGVTEFEARYGTLPPASQRWDRILQASGMKRAKPSPTSAQTPDQASLHAFADSLERDLDAPSPMHEGDQTRASSRKRSRSDRAVTGPSTQQSFEVRVPEQQDALHLPLSWRVKRPRTRIGGGLPDPGTPIAADLAASSTVMWEQDAAPFAGAADDFPAFNEEELAWLMELLPQSGSVGGTI

SEQ ID NO: 20 - DNA, 4341 bp, Artificial Sequence
  Synthetic construct
atggatcccattcgttcgcgcacgccaagtcctgcccgcgagcttctgcccggaccccaaccggatagggttcagccgactgcagatcgggggggggctccgcctgctggcggccccctggatggcttgcccgctcggcggacgatgtcccggacccggctgccatctccccctgcgccctcgcctgcgttctcggcgggcagcttcagcgatctgctccgtcagttcgatccgtcgcttcttgatacatcgcttcttgattcgatgcctgccgtcggcacgccgcatacagcggctgccccagcagagtgcgatgaggtgcaatcgggtctgcgtgcagccgatgacccgccacccaccgtgcgtgtcgctgtcactgcggcgcggccgccgcgcgccaagccggccccgcgacggcgtgcggcgcaaccctccgacgcttcgccggccgcgcaggtggatctacgcacgctcggctacagtcagcagcagcaagagaagatcaaaccgaaggtgcgttcgacagtggcgcagcaccacgaggcactggtgggccatgggtttacacacgcgcacatcgttgcgctcagccaacacccggcagcgttagggaccgttgctgtcacgtatcaggacataatcagggcgttgccagaggcgacacacgaagacatcgttggcgtcggcaaacagtggtccggcgcacgcgctctggaggccttgctcacggaggcgggggagttgagaggtccgccgttacagttggacacaggccaacttctcaagattgcaaaacgtggcggcgtgaccgcagtggaggcagtgcatgcatggcgcaatgcactgacgggtgcccccctgaacctgaccccggaccaagtggtggccatcgccagcaatattggcggcaagcaggcgctggagacggtacagcggctgttgccggtgctgtgccaggaccatggcctgaccccggaccaggtcgtggccatcgccagccatggcggcggcaagcaggcgctggagacggtgcagcggctgttgccggtgctgtgccaggaccatggcctgaccccggaccaggtggtggccatcgccagcaatattggcggcaagcaggcgctagagacggtgcagcggctgttgccggtgctgtgccaggcccatggcctgaccccggaccaggtcgtggccatcgccagcaatattggcggcaagcaggcgctggagacggtgcagcggctgttgccggtgctgtgccaggaccatggcctgaccccggcccaggtggtggccatcgccagcaatagtggcggcaagcaggcgctggagacggtgcagcggctgttgccggtgctgtgccaggaccatggcctgaccccggaccaagtcgtggccatcgccagccacgatggcggcaagcaggcgctggagacgctgcagcggctgttgccggtgctgtgccaggaccatggcctgaccccggaccaggtcgtggccatcgccaacaataacggcggcaagcaggcgctggagacgctgcagcggctgttgccggtgctgtgccaggaccatggcctgaccccggaccaagtggtggccatcgccagccacgatggcggcaagcaggcgctggagacggtgcagcggctgttgccggtgctgtgccaggaccatggcctgaccccggaccaggtggtggccatcgccagccacgatggcggcaagcaggcgctggagacggtgcagcggctgttgccggtgctgtgccaggaccatggcctgaccccggcccaagtggtggccatcgccagccacgatggcggcaagcaggcgctggagacggtgcagcggctgttgccggtgctgtgccaggaccatggcctgaccccggaccaggtggtggccatcgccagcaatagcggcggcaagcaggcgctggagacggtacagcggctgttgccggtgctgtgccaggaccatggactgaccccggaccaggtcgtggccatcgccagcaatggcggcaagcaggcgctggagacggtacagcggctgttgccggtgctgtgccaggaccatggcctgaccccggaccaggtcgtggccatcgccagcaatggcggcaagcaggcgctggagacggtgcagcggctgttgccggtacagcggctgttgccggtgctgtgccaggaccatggcctgacccaggaccaggtggtggccatcgccagccacgatggcggcaagcaggcgctggagacggtgcagcggctgttgccggtgctgtgccaggaccatggcctgaccccggaccaagtggtggccatcgccagccacgatggcggcaaacaggcgctggagacggtgcagcggctgttgccggtgctgtgccaggaccatggcctgaccccggaccaggtggtggccatcgccagcaatagtggcggcaagcaggcgctggagacggtgcagcggctgttgccggtgctgtgccaggaccatggcctgaccccggaccaagtggtggccatcgccagcaatagtggcggcaagcaggcgctggagacggtgcagcggctgttgccggtgctgtgccaggaccatggcctgaccccggaccaggtggtggccatcgccagcaataacggcggcaagcaggcgctggagacggtgcagcggctgttgccggtgctgtgccaggaccatggcctgaccccggaccaggtcgtggccatcgccaacaataacggcggcaagcaggcgctggagacggtgcagcggctgttgccggtgctgtgccaggaccatggcctgaccccggcgcaggtggtggccatcgccagcaatattggcggcaagcaggcgctggagacggtgcagcggctgttgccggtgctgtgccaggaccatggcctgaccctggaccaggtggtggccattgccagcaatggcggcagcaaacaggcgctagagacggtgcagcggctgttgccggtgctgtgccaggaccatggcctgaccccggaccaagtggtggccatcgccaacaataacggcggcaagcaggcgctggagacggtgcagcggctgttgccggtgctgtgccaggaccatggcctgaccccggaccaggtcgtggccatcgccagcaatattggcggcaagcaggcgctggagacggtgcagcggctgttgccggtgctgtgccaggaccatggcctgaccctggaccaggtggtggccatcgccagcaatggcggcaagcaggcgctggagacggtgcagcggctgttgccggtgctgtgccaggaccatggcctgaccccgaaccaggtggtggccatcgccagcaatagtggcggcaagcaggcgctggagacggtgcagcggctgttgccggtgctgtgccaggaccatggcctgaccccgaaccaggtggtggccatcgccagcaatggcggcaagcaggcgctggagagcattgttgcccagttatctcgccctgatccggcgttggccgcgttgaccaacgaccacctcgtcgccttggcctgcctcggcggacgtcctgccctggatgcagtgaaaaagggattgccgcacgcgccggaattgatcagaagaatcaatcgccgcattcccgaacgcacgtcccatcgcgttcccgacctcgcgcacgtggttcgcgtgcttggttttttccagagccactcccacccagcgcaagcattcgatgacgccatgacgcagttcgagatgagcaggcacggcttggtacagctctttcgcagagtgggcgtcaccgaattcgaagcccgctacggaacgctccccccagcctcgcagcgttgggaccgtatcctccaggcatcagggatgaaaagggccaaaccgtcccctacttcagctcaaacaccggatcaggcgtctttgcatgcattcgccgattcgctggagcgtgaccttgatgcgcccagcccaatgcacgagggagatcagacgcgggcaagcagccgtaaacggtcccgatcggatcgtgctgtcaccggcccctccacacagcaatctttcgaggtgcgcgttcccgaacagcaagatgcgctgcatttgcccctcagctggagggtaaaacgcccgcgtaccaggatcgggggcggcctcccggatcctggtacgcccatcgctgccgacctggcagcgtccagcaccgtgatgtgggaacaagatgcggcccccttcgcaggggcagcggatgatttcccggcattcaacgaagaggagctcgcatggttgatggagctattgcctcagtcaggctcagtcggagggacgatctga

SEQ ID NO: 21 - protein, 1263 aa, Artificial Sequence
  Synthetic construct
MLIGYVRVSTNDQNTDLQRNALVCAGCEQIFEDKLSGTRTDRPGLKRALKRLQKGDTLVVWKLDRLGRSMKHLISLVGELRERGINFRSLTDSIDTSSPMGRFFFYVMGALAEMERELIIERTMAGLAAARNKGRIGGRPRKSGSGSPRQFDPSLLDTSLLDSMPAVGTPHTAAAPAECDEVQSGLRAADDPPPTVRVAVTAARPPRAKPAPRRRAAQPSDASPAAQVDLRTLGYSQQQQEKIKPKVRSTVAQHHEALVGHGFTHAHIVALSQHPAALGTVAVTYQDIIRALPEATHEDIVGVGKQWSGARALEALLTEAGELRGPPLQLDTGQLLKIAKRGGVTAVEAVHAWRNALTGAPLNLTPDQVVAIASNIGGKQALETVQRLLPVLCQDHGLTPDQVVAIASHGGGKQALETVQRLLPVLCQDHGLTPDQVVAIASNIGGKQALETVQRLLPVLCQAHGLTPDQVVAIASNIGGKQALETVQRLLPVLCQDHGLTPAQVVAIASNSGGKQALETVQRLLPVLCQDHGLTPDQVVAIASHDGGKQALETLQRLLPVLCQDHGLTPDQVVAIANNNGGKQALETLQRLLPVLCQDHGLTPDQVVAIASHDGGKQALETVQRLLPVLCQDHGLTPDQVVAIASHDGGKQALETVQRLLPVLCQDHGLTPAQVVAIASHDGGKQALETVQRLLPVLCQDHGLTPDQVVAIASNSGGKQALETVQRLLPVLCQDHGLTPDQVVAIASNGGKQALETVQRLLPVLCQDHGLTPDQVVAIASNGGKQALETVQRLLPVQRLLPVLCQDHGLTQDQVVAIASHDGGKQALETVQRLLPVLCQDHGLTPDQVVAIASHDGGKQALETVQRLLPVLCQDHGLTPDQVVAIASNSGGKQALETVQRLLPVLCQDHGLTPDQVVAIASNSGGKQALETVQRLLPVLCQDHGLTPDQVVAIASNNGGKQALETVQRLLPVLCQDHGLTPDQVVAIANNNGGKQALETVQRLLPVLCQDHGLTPAQVVAIASNIGGKQALETVQRLLPVLCQDHGLTLDQVVAIASNGGSKQALETVQRLLPVLCQDHGLTPDQVVAIANNNGGKQALETVQRLLPVLCQDHGLTPDQVVAIASNIGGKQALETVQRLLPVLCQDHGLTLDQVVAIASNGGKQALETVQRLLPVLCQDHGLTPNQVVAIASNSGGKQALETVQRLLPVLCQDHGLTPNQVVAIASNGGKQALESIVAQLSRPDPALAALTNDHLVALACLG

SEQ ID NO: 22 - protein, 1250 aa, Artificial Sequence
  Synthetic construct
MLIGYVRVSTNDQNTDLQRNALVCAGCEQIFEDKLSGTRTDRPGLKRALKRLQKGDTLVVWKLDRLGRSMKHLISLVGELRERGINFRSLTDSIDTSSPMGRFFFYVMGALAEMERELIIERTMAGLAAARNKGRIGGRPRKSGSGSPDSMPAVGTPHTAAAPAECDEVQSGLRAADDPPPTVRVAVTAARPPRAKPAPRRRAAQPSDASPAAQVDLRTLGYSQQQQEKIKPKVRSTVAQHHEALVGHGFTHAHIVALSQHPAALGTVAVTYQDIIRALPEATHEDIVGVGKQWSGARALEALLTEAGELRGPPLQLDTGQLLKIAKRGGVTAVEAVHAWRNALTGAPLNLTPDQVVAIASNIGGKQALETVQRLLPVLCQDHGLTPDQVVAIASHGGGKQALETVQRLLPVLCQDHGLTPDQVVAIASNIGGKQALETVQRLLPVLCQAHGLTPDQVVAIASNIGGKQALETVQRLLPVLCQDHGLTPAQVVAIASNSGGKQALETVQRLLPVLCQDHGLTPDQVVAIASHDGGKQALETLQRLLPVLCQDHGLTPDQVVAIANNNGGKQALETLQRLLPVLCQDHGLTPDQVVAIASHDGGKQALETVQRLLPVLCQDHGLTPDQVVAIASHDGGKQALETVQRLLPVLCQDHGLTPAQVVAIASHDGGKQALETVQRLLPVLCQDHGLTPDQVVAIASNSGGKQALETVQRLLPVLCQDHGLTPDQVVAIASNGGKQALETVQRLLPVLCQDHGLTPDQVVAIASNGGKQALETVQRLLPVQRLLPVLCQDHGLTQDQVVAIASHDGGKQALETVQRLLPVLCQDHGLTPDQVVAIASHDGGKQALETVQRLLPVLCQDHGLTPDQVVAIASNSGGKQALETVQRLLPVLCQDHGLTPDQVVAIASNSGGKQALETVQRLLPVLCQDHGLTPDQVVAIASNNGGKQALETVQRLLPVLCQDHGLTPDQVVAIANNNGGKQALETVQRLLPVLCQDHGLTPAQVVAIASNIGGKQALETVQRLLPVLCQDHGLTLDQVVAIASNGGSKQALETVQRLLPVLCQDHGLTPDQVVAIANNNGGKQALETVQRLLPVLCQDHGLTPDQVVAIASNIGGKQALETVQRLLPVLCQDHGLTLDQVVAIASNGGKQALETVQRLLPVLCQDHGLTPNQVVAIASNSGGKQALETVQRLLPVLCQDHGLTPNQVVAIASNGGKQALESIVAQLSRPDPALAALTNDHLVALACLG

SEQ ID NO: 23 - protein, 1216 aa, Artificial Sequence
  Synthetic construct
MLIGYVRVSTNDQNTDLQRNALVCAGCEQIFEDKLSGTRTDRPGLKRALKRLQKGDTLVVWKLDRLGRSMKHLISLVGELRERGINFRSLTDSIDTSSPMGRFFFYVMGALAEMERELIIERTMAGLAAARNKGRIGGRPRKSGSGSTVRVAVTAARPPRAKPAPRRRAAQPSDASPAAQVDLRTLGYSQQQQEKIKPKVRSTVAQHHEALVGHGFTHAHIVALSQHPAALGTVAVTYQDIIRALPEATHEDIVGVGKQWSGARALEALLTEAGELRGPPLQLDTGQLLKIAKRGGVTAVEAVHAWRNALTGAPLNLTPDQVVAIASNIGGKQALETVQRLLPVLCQDHGLTPDQVVAIASHGGGKQALETVQRLLPVLCQDHGLTPDQVVAIASNIGGKQALETVQRLLPVLCQAHGLTPDQVVAIASNIGGKQALETVQRLLPVLCQDHGLTPAQVVAIASNSGGKQALETVQRLLPVLCQDHGLTPDQVVAIASHDGGKQALETLQRLLPVLCQDHGLTPDQVVAIANNNGGKQALETLQRLLPVLCQDHGLTPDQVVAIASHDGGKQALETVQRLLPVLCQDHGLTPDQVVAIASHDGGKQALETVQRLLPVLCQDHGLTPAQVVAIASHDGGKQALETVQRLLPVLCQDHGLTPDQVVAIASNSGGKQALETVQRLLPVLCQDHGLTPDQVVAIASNGGKQALETVQRLLPVLCQDHGLTPDQVVAIASNGGKQALETVQRLLPVQRLLPVLCQDHGLTQDQVVAIASHDGGKQALETVQRLLPVLCQDHGLTPDQVVAIASHDGGKQALETVQRLLPVLCQDHGLTPDQVVAIASNSGGKQALETVQRLLPVLCQDHGLTPDQVVAIASNSGGKQALETVQRLLPVLCQDHGLTPDQVVAIASNNGGKQALETVQRLLPVLCQDHGLTPDQVVAIANNNGGKQALETVQRLLPVLCQDHGLTPAQVVAIASNIGGKQALETVQRLLPVLCQDHGLTLDQVVAIASNGGSKQALETVQRLLPVLCQDHGLTPDQVVAIANNNGGKQALETVQRLLPVLCQDHGLTPDQVVAIASNIGGKQALETVQRLLPVLCQDHGLTLDQVVAIASNGGKQALETVQRLLPVLCQDHGLTPNQVVAIASNSGGKQALETVQRLLPVLCQDHGLTPNQVVAIASNGGKQALESIVAQLSRPDPALAALTNDHLVALACLG

SEQ ID NO: 24 - protein, 1204 aa, Artificial Sequence
  Synthetic construct
MLIGYVRVSTNDQNTDLQRNALVCAGCEQIFEDKLSGTRTDRPGLKRALKRLQKGDTLVVWKLDRLGRSMKHLISLVGELRERGINFRSLTDSIDTSSPMGRFFFYVMGALAEMERELIIERTMAGLAAARNKGRIGGRPRKSGSGSTVRVAVTAARPPHAVAGPAAQVDLRTLGYSQQQQEKIKPKVRSTVAQHHEALVGHGFTHAHIVALSQHPAALGTVAVTYQDIIRALPEATHEDIVGVGKQWSGARALEALLTEAGELRGPPLQLDTGQLLKIAKRGGVTAVEAVHAWRNALTGAPLNLTPDQVVAIASNIGGKQALETVQRLLPVLCQDHGLTPDQVVAIASHGGGKQALETVQRLLPVLCQDHGLTPDQVVAIASNIGGKQALETVQRLLPVLCQAHGLTPDQVVAIASNIGGKQALETVQRLLPVLCQDHGLTPAQVVAIASNSGGKQALETVQRLLPVLCQDHGLTPDQVVAIASHDGGKQALETLQRLLPVLCQDHGLTPDQVVAIANNNGGKQALETLQRLLPVLCQDHGLTPDQVVAIASHDGGKQALETVQRLLPVLCQDHGLTPDQVVAIASHDGGKQALETVQRLLPVLCQDHGLTPAQVVAIASHDGGKQALETVQRLLPVLCQDHGLTPDQVVAIASNSGGKQALETVQRLLPVLCQDHGLTPDQVVAIASNGGKQALETVQRLLPVLCQDHGLTPDQVVAIASNGGKQALETVQRLLPVQRLLPVLCQDHGLTQDQVVAIASHDGGKQALETVQRLLPVLCQDHGLTPDQVVAIASHDGGKQALETVQRLLPVLCQDHGLTPDQVVAIASNSGGKQALETVQRLLPVLCQDHGLTPDQVVAIASNSGGKQALETVQRLLPVLCQDHGLTPDQVVAIASNNGGKQALETVQRLLPVLCQDHGLTPDQVVAIANNNGGKQALETVQRLLPVLCQDHGLTPAQVVAIASNIGGKQALETVQRLLPVLCQDHGLTLDQVVAIASNGGSKQALETVQRLLPVLCQDHGLTPDQVVAIANNNGGKQALETVQRLLPVLCQDHGLTPDQVVAIASNIGGKQALETVQRLLPVLCQDHGLTLDQVVAIASNGGKQALETVQRLLPVLCQDHGLTPNQVVAIASNSGGKQALETVQRLLPVLCQDHGLTPNQVVAIASNGGKQALESIVAQLSRPDPALAALTNDHLVALACLG

SEQ ID NO: 25 - protein, 1190 aa, Artificial Sequence
  Synthetic construct
MLIGYVRVSTNDQNTDLQRNALVCAGCEQIFEDKLSGTRTDRPGLKRALKRLQKGDTLVVWKLDRLGRSMKHLISLVGELRERGINFRSLTDSIDTSSPMGRFFFYVMGALAEMERELIIERTMAGLAAARNKGRIGGRPRKSGSGSPASPAAQVDLRTLGYSQQQQEKIKPKVRSTVAQHHEALVGHGFTHAHIVALSQHPAALGTVAVTYQDIIRALPEATHEDIVGVGKQWSGARALEALLTEAGELRGPPLQLDTGQLLKIAKRGGVTAVEAVHAWRNALTGAPLNLTPDQVVAIASNIGGKQALETVQRLLPVLCQDHGLTPDQVVAIASHGGGKQALETVQRLLPVLCQDHGLTPDQVVAIASNIGGKQALETVQRLLPVLCQAHGLTPDQVVAIASNIGGKQALETVQRLLPVLCQDHGLTPAQVVAIASNSGGKQALETVQRLLPVLCQDHGLTPDQVVAIASHDGGKQALETLQRLLPVLCQDHGLTPDQVVAIANNNGGKQALETLQRLLPVLCQDHGLTPDQVVAIASHDGGKQALETVQRLLPVLCQDHGLTPDQVVAIASHDGGKQALETVQRLLPVLCQDHGLTPAQVVAIASHDGGKQALETVQRLLPVLCQDHGLTPDQVVAIASNSGGKQALETVQRLLPVLCQDHGLTPDQVVAIASNGGKQALETVQRLLPVLCQDHGLTPDQVVAIASNGGKQALETVQRLLPVQRLLPVLCQDHGLTQDQVVAIASHDGGKQALETVQRLLPVLCQDHGLTPDQVVAIASHDGGKQALETVQRLLPVLCQDHGLTPDQVVAIASNSGGKQALETVQRLLPVLCQDHGLTPDQVVAIASNSGGKQALETVQRLLPVLCQDHGLTPDQVVAIASNNGGKQALETVQRLLPVLCQDHGLTPDQVVAIANNNGGKQALETVQRLLPVLCQDHGLTPAQVVAIASNIGGKQALETVQRLLPVLCQDHGLTLDQVVAIASNGGSKQALETVQRLLPVLCQDHGLTPDQVVAIANNNGGKQALETVQRLLPVLCQDHGLTPDQVVAIASNIGGKQALETVQRLLPVLCQDHGLTLDQVVAIASNGGKQALETVQRLLPVLCQDHGLTPNQVVAIASNSGGKQALETVQRLLPVLCQDHGLTPNQVVAIASNGGKQALESIVAQLSRPDPALAALTNDHLVALACLG

SEQ ID NO: 26 - protein, 841 aa, Artificial Sequence
  Synthetic construct
MLIGYVRVSTNDQNTDLQRNALVCAGCEQIFEDKLSGTRTDRPGLKRALKRLQKGDTLVVWKLDRLGRSMKHLISLVGELRERGINFRSLTDSIDTSSPMGRFFFYVMGALAEMERELIIERTMAGLAAARNKGRIGGRPRKSGSGSPALRPPRAKPAPRRRAAQPSDASPAAQVDLRTLGYSQQQQEKIKPKVRSTVAQHHEALVGHGFTHAHIVALSQHPAALGTVAVTYQHIITALPEATHEDIVGVGKQWSGARALEALLTDAGELRGPPLQLDTGQLVKIAKRGGVTAMEAVHASRNALTGAPLNLTPDQVVAIASNIGGKQALETVQRLLPVLCQDHGLTPDQVVAIASNGGGKQALETVQRLLPVLCQDHGLTPDQVVAIASNIGGKQALETVQRLLPVLCQDHGLTPDQVVAIASNIGGKQALETVQRLLPVLCQDHGLTPDQVVAIASNIGGKQALETVQRLLPVLCQDHGLTPDQVVAIASHDGGKQALETVQRLLPVLCQDHGLTPDQVVAIASHDGGKQALETVQRLLPVLCQDHGLTPDQVVAIASHDGGKQALETVQRLLPVLCQDHGLTPDQVVAIASHDGGKQALETVQRLLPVLCQDHGLTPDQVVAIASHDGGKQALETVQRLLPVLCQDHGLTPDQVVAIASNGGGKQALETVQRLLPVLCQDHGLTPDQVVAIASHDGGKQALETVQRLLPVLCQDHGLTPDQVVAIASHDGGKQALETVQRLLPVLCQDHGLTPDQVVAIASNIGGKQALETVQRLLPVLCQDHGLTPDQVVAIASNIGGKQALESIVAQLSRPDPALAALTNDHLVALACLGPKKKRKV

SEQ ID NO: 27 - DNA, 2523 bp, Artificial Sequence
  Synthetic construct
atgctgattggctatgtaagggtatcaacaaatgaccagaatacagacctgcaacgaaacgctcttgtttgtgcaggatgtgaacaaatatttgaagataaattaagcggaacaaggacagaccgaccgggattaaaacgcgctttaaagcgccttcaaaaaggtgacacactggttgtctggaaactggatcgcctcgggcgaagcatgaaacatttgatttctctcgtaggggaattacgagagcgagggattaattttcgcagtcttactgacagtattgatacgtcatctccaatggggcgttttttcttctacgttatgggtgccctggctgaaatggaacgagaactaattatcgagcgaacgatggctggacttgctgccgccagaaataaaggccgtattggaggtcgcccgcgtaaatcggggtctggatcccccgcgcggccgccgcgcgccaagccggccccgcgacggcgtgctgcgcaaccctccgacgcttcgccggccgcgcaggtggatctacgcacgctcggctacagtcagcagcagcaagagaagatcaaaccgaaggtgcgttcgacagtggcgcagcaccacgaggcactggtgggccatgggtttacacacgcgcacatcgttgcgctcagccaacacccggcagcgttagggaccgtcgctgtcacgtatcagcacataatcacggcgttgccagaggcgacacacgaagacatcgttggcgtcggcaaacagtggtccggcgcacgcgccctggaggccttgctcacggatgcgggggagttgagaggtccgccgttacagttggacacaggccaacttgtgaagattgcaaaacgtggcggcgtgaccgcaatggaggcagtgcatgcatcgcgcaatgcactgacgggtgcccccctggagctgactccggaccaagtggtggctatcgccagcaacattggcggcaagcaagcgctcgaaacggtgcagcggctgttgccggtgctgtgccaggaccatggcctgactccggaccaagtggtggctatcgccagcaacggtggcggcaagcaagcgctcgaaacggtgcagcggctgttgccggtgctgtgccaggaccatggcctgactccggaccaagtggtggctatcgccagcaacattggcggcaagcaagcgctcgaaacggtgcagcggctgttgccggtgctgtgccaggaccatggcctgactccggaccaagtggtggctatcgccagcaacattggcggcaagcaagcgctcgaaacggtgcagcggctgttgccggtgctgtgccaggaccatggcctgactccggaccaagtggtggctatcgccagcaacattggcggcaagcaagcgctcgaaacggtgcagcggctgttgccggtgctgtgccaggaccatggcctgactccggaccaagtggtggctatcgccagccacgatggcggcaagcaagcgctcgaaacggtgcagcggctgttgccggtgctgtgccaggaccatggcctgactccggaccaagtggtggctatcgccagccacgatggcggcaagcaagcgctcgaaacggtgcagcggctgttgccggtgctgtgccaggaccatggcctgactccggaccaagtggtggctatcgccagccacgatggcggcaagcaagcgctcgaaacggtgcagcggctgttgccggtgctgtgccaggaccatggcctgactccggaccaagtggtggctatcgccagccacgatggcggcaagcaagcgctcgaaacggtgcagcggctgttgccggtgctgtgccaggaccatggcctgactccggaccaagtggtggctatcgccagccacgatggcggcaagcaagcgctcgaaacggtgcagcggctgttgccggtgctgtgccaggaccatggcctgaccccggaccaagtggtggctatcgccagcaacggtggcggcaagcaagcgctcgaaacggtgcagcggctgttgccggtgctgtgccaggaccatggcctgactccggaccaagtggtggctatcgccagccacgatggcggcaagcaagcgctcgaaacggtgcagcggctgttgccggtgctgtgccaggaccatggcctgactccggaccaagtggtggctatcgccagccacgatggcggcaagcaagcgctcgaaacggtgcagcggctgttgccggtgctgtgccaggaccatggcctgaccccggaccaagtggtggctatcgccagcaacattggcggcaagcaagcgctcgaaacggtgcagcggctgttgccggtgctgtgccaggaccatggcctgaccccggaccaagtggtggctatcgccagcaacattggcggcaagcaagcgctcgaaagcattgtggcccagctgagccggcctgatccggcgttggccgcgttgaccaacgaccacctcgtcgccttggcctgcctcggccccaagaagaagcgcaaggtgtag

SEQ ID NO: 28 - protein, 841 aa, Artificial Sequence; identical to SEQ ID NO: 26
  Synthetic construct

SEQ ID NO: 29 - protein, 134 aa, Artificial Sequence
  Synthetic construct
VDLRTLGYSQQQQEKIKPKVRSTVAQHHEALVGHGFTHAHIVALSQHPAALGTVAVTYQHIITALPEATHEDIVGVGKQWSGARALEALLTDAGELRGPPLQLDTGQLVKIAKRGGVTAMEAVHASRNALTGAP

SEQ ID NO: 30 - protein, 34 aa, Artificial Sequence
  Synthetic construct
LTDGQLVKIAKRGGVTAMEAVHASRNALTGAPLN

SEQ ID NO: 31 - protein, 30 aa, Artificial Sequence
  Synthetic construct
THEDIVGVGKQWSGARALEALLTDAGELRG

SEQ ID NO: 32 - protein, 34 aa, Artificial Sequence
  Synthetic construct
  misc_feature (12)..(13): Xaa can be any naturally occurring amino acid
LTPDQVVAIASXXGGKQALETVQRLLPVLCQDHG

SEQ ID NO: 33 - protein, 15 aa, Artificial Sequence
  Synthetic construct
DIVGVKQWSGARALE

SEQ ID NO: 34 - protein, 15 aa, Artificial Sequence
  Synthetic construct
DIVGVKSRSGARALE

SEQ ID NO: 35 - protein, 15 aa, Artificial Sequence
  Synthetic construct
DIVGVKRGAGARALE

SEQ ID NO: 36 - protein, 14 aa, Artificial Sequence
  Synthetic construct
DIVGVKYHGARALE

SEQ ID NO: 37 - DNA, 21 bp, Artificial Sequence
  Synthetic construct
ataaaccccctccaaccaggc

SEQ ID NO: 38 - DNA, 71 bp, Artificial Sequence
  Synthetic construct
aagaaggtcttcattacacctgcagctctcattttccatacagtcagtatcaattctggaagaatttccag

SEQ ID NO: 39 - protein, 7 aa, Artificial Sequence
  Synthetic construct
  misc_feature (1)..(3): Xaa can be any naturally occurring amino acid
XXXSGAR

SEQ ID NO: 40 - DNA, 18 bp, Artificial Sequence
  Synthetic construct
gtcttcattacacctgca

SEQ ID NO: 41 - DNA, 18 bp, Artificial Sequence
  Synthetic construct
cttcattacacctgcagc

SEQ ID NO: 42 - DNA, 18 bp, Artificial Sequence
  Synthetic construct
ttcattacacctgcagct

SEQ ID NO: 43 - DNA, 18 bp, Artificial Sequence
  Synthetic construct
acctgcagctctcatttt

SEQ ID NO: 44 - DNA, 16 bp, Artificial Sequence
  Synthetic construct
gtcagtcatagttaag

SEQ ID NO: 45 - DNA, 18 bp, Artificial Sequence
  Synthetic construct
tcagtcatagttaagacc

SEQ ID NO: 46 - DNA, 19 bp, Artificial Sequence
  Synthetic construct
tcatagttaagaccttctt

SEQ ID NO: 47 - DNA, 17 bp, Artificial Sequence
  Synthetic construct
agttaagaccttcttaa

SEQ ID NO: 48 - protein, 159 aa, Artificial Sequence
  Synthetic construct
  misc_feature (104)..(107): Xaa can be any naturally occurring amino acid
PRPPRAKPAPRRRAAQPSDASPAAQVDLRTLGYSQQQQEKIKPKVRSTVAQHHEALVGHGFTHAHIVALSQHPAALGTVAVTYQHIITALPEATHEDIVGVGKXXXXARALEALLTDAGELRGPPLQLDTGQLVKIAKRGGVTAMEAVHASRNALTGAP

SEQ ID NO: 49 - protein, 134 aa, Artificial Sequence
  Synthetic construct
  misc_feature (79)..(82): Xaa can be any naturally occurring amino acid
VDLRTLGYSQQQQEKIKPKVRSTVAQHHEALVGHGFTHAHIVALSQHPAALGTVAVTYQHIITALPEATHEDIVGVGKXXXXARALEALLTDAGELRGPPLQLDTGQLVKIAKRGGVTAMEAVHASRNALTGAP

SEQ ID NO: 50 - protein, 134 aa, Artificial Sequence
  Synthetic construct
VDLRTLGYSQQQQEKIKPKVRSTVAQHHEALVGHGFTHAHIVALSQHPAALGTVAVKYQDMIAALPEATHEAIVGVGKQWSGARALEALLTVAGELRGPPLQLDTGQLLKIAKRGGVTAVEAVHAWRNALTGAP

SEQ ID NO: 51 - protein, 80 aa, Artificial Sequence
  Synthetic construct
NDHLVALACLGGRPAMDAVKKGLPHAPELIRRVNRRIGERTSHRVADYAQVVRVLEFFQCHSHPAYAFDEAMTQFGMSGQ

SEQ ID NO: 52 - protein, 46 aa, Artificial Sequence
  Synthetic construct
NDHLVALACLGGRPAMDAVKKGLPHAPELIRRVNRRIGERTSHRVA

SEQ ID NO: 53 - protein, 10 aa, Artificial Sequence
  Synthetic construct
NDHLVALACL

SEQ ID NO: 54 - protein, 135 aa, Artificial Sequence
  Synthetic construct
QVDLRTLGYSQQQQEKIKPKVRSTVAQHHEALVGHGFTHAHIVALSQHPAALGTVAVTYQHIITALPEATHEDIVGVGKSRSGARALEALLTDAGELRGPPLQLDTGQLVKIAKRGGVTAMEAVHASRNALTGAP

SEQ ID NO: 55 - protein, 132 aa, Artificial Sequence
  Synthetic construct
MAALGYSREQIRKLKQESLSGVAKYHAPLTRHGFTHTDICRISRRWQSLRMVAKNYPKLIAALPDLTRTHIVDIARQRSGDLALEALLPVATALAAAPLRLRASQIAIIAQCGERPAILALHRLRRKLTGAP

SEQ ID NO: 56 - protein, 180 aa, Artificial Sequence
  Synthetic construct
MLIGYVRVSTNDQNTDLQRNALVCAGCEQIFEDKLSGTRTDRPGLKRALKRLQKGDTLVVWKLDRLGRSMKHLISLVGELRERGINFRSLTDSIDTSSPMGRFFFYVMGALAEMERELIIERTMAGLAAARNKGRIGGRPPKLTKAEWEQAGRLLAQGIPRKQVALIYDVALSTLYKKHP

SEQ ID NO: 57 - protein, 144 aa, Artificial Sequence
  Synthetic construct
MLIGYVRVSTNDQNTDLQRNALVCAGCEQIFEDKLSGTRTDRPGLKRALKRLQKGDTLVVWKLDRLGRSMKHLISLVGELRERGINFRSLTDSIDTSSPMGRFFFYVMGALAEMERELIIERTMAGLAAARNKGRIGGRPPKSG

SEQ ID NO: 58 - protein, 143 aa, Artificial Sequence
  Synthetic construct
MLIGYVRVSTNDQNTDLQRNALVCAGCEQIFEDKLSGTRTDRPGLKRALKRLQKGDTLVVWKLDRLGRSMKHLISLVGELRERGINFRSLTDSIDTSSPMGRFFFYVMGALAEMERELIIERTMAGIAAARNKGRRFGRPPKS

SEQ ID NO: 59 - protein, 144 aa, Artificial Sequence
  Synthetic construct
MLIGYVRVSTNDQNTDLQRNALVCAGCEQIFEDKLSGTRTDRPGLKRALKRLQKGDTLVVWKLDRLGRSMKHLISLVGELRERGINFRSLTDSIDTSSPMGRFFFYVMGALAEMERELILERVMAGIAAARNKGRRWGRPPKSG

SEQ ID NO: 60 - protein, 144 aa, Artificial Sequence
  Synthetic construct
MLIGYVRVSTNDQNTDLQRNALVCAGCEQIFEDKLSGTRTDRPGLKRALKRLQKGDTLVVWKLDRLGRSMKHLISLVGELRERGINFRSLTDSIDTSSPMGRFFFYVMGALAEMERELIIERVMAGLAAARNKGRRFGRPPKSG

SEQ ID NO: 61 - protein, 144 aa, Artificial Sequence
  Synthetic construct
MLIGYVRVSTNDQNTDLQRNALVCAGCEQIFEDKLSGTRTDRPGLKRALKRLQKGDTLVVWKLDRLGRSMKHLISLVGELRERGINFRSLTDSIDTSSPMGRFFFYVMGALAEMERLSILERPMAGHAAARNKGRRFGRPPKSG

SEQ ID NO: 62 - protein, 144 aa, Artificial Sequence
  Synthetic construct
MLIGYVRVSTNDQNTDLQRNALVCAGCEQIFEDKLSGTRTDRPGLKRALKRLQKGDTLVVWKLDRLGRSMKHLISLVGELRERGINFRSLTDSIDTSSPMGRFFFYVMGALAEMERELIIERTSAGRAAAINKGRIMGRPRKSG

SEQ ID NO: 63 - protein, 267 aa, Artificial Sequence
  Synthetic construct
MLIGYVRVSTNDQNTDLQRNALVCAGCEQIFEDKLSGTRTDRPGLKRALKRLQKGDTLVVWKLDRLGRSMKHLISLVGELRERGINFRSLTDSIDTSSPMGRFFFYVMGALAEMERELIIERTMAGLAAARNKGRIGGRPPKSGTGEKPYKCPECGKSFSTSGNLVRHQRTHTGEKPYKCPECGKSFSQSGDLRRHQRTHTGEKPYKCPECGKSFSTSGNLVRHQRTHTGEKPYKCPECGKSFSTSGELVRHQRTHTGKKTSGQAGQ

SEQ ID NO: 64 - protein, 267 aa, Artificial Sequence
  Synthetic construct
MLIGYVRVSTNDQNTDLQRNALVCAGCEQIFEDKLSGTRTDRPGLKRALKRLQKGDTLVVWKLDRLGRSMKHLISLVGELRERGINFRSLTDSIDTSSPMGRFFFYVMGALAEMERELIIERTMAGLAAARNKGRIGGRPPKSGTGEKPYKCPECGKSFSHRTTLTNHQRTHTGEKPYKCPECGKSFSQSGDLRRHQRTHTGEKPYKCPECGKSFSQSGDLRRHQRTHTGEKPYKCPECGKSFSQSGDLRRHQRTHTGKKTSGQAGQ

SEQ ID NO: 65 - protein, 267 aa, Artificial Sequence
  Synthetic construct
MLIGYVRVSTNDQNTDLQRNALVCAGCEQIFEDKLSGTRTDRPGLKRALKRLQKGDTLVVWKLDRLGRSMKHLISLVGELRERGINFRSLTDSIDTSSPMGRFFFYVMGALAEMERELIIERTMAGLAAARNKGRIGGRPPKSGTGEKPYKCPECGKSFSQSGDLRRHQRTHTGEKPYKCPECGKSFSQRAHLERHQRTHTGEKPYKCPECGKSFSTSGNLVRHQRTHTGEKPYKCPECGKSFSRSDELVRHQRTHTGKKTSGQAGQ

SEQ ID NO: 66 - protein, 267 aa, Artificial Sequence
  Synthetic construct
MLIGYVRVSTNDQNTDLQRNALVCAGCEQIFEDKLSGTRTDRPGLKRALKRLQKGDTLVVWKLDRLGRSMKHLISLVGELRERGINFRSLTDSIDTSSPMGRFFFYVMGALAEMERELIIERTMAGLAAARNKGRIGGRPPKSGTGEKPYKCPECGKSFSRSDKLVRHQRTHTGEKPYKCPECGKSFSRKDNLKNHQRTHTGEKPYKCPECGKSFSTSGELVRHQRTHTGEKPYKCPECGKSFSRSDKLVRHQRTHTGKKTSGQAGQ

SEQ ID NO: 67 - protein, 267 aa, Artificial Sequence
  Synthetic construct
MLIGYVRVSTNDQNTDLQRNALVCAGCEQIFEDKLSGTRTDRPGLKRALKRLQKGDTLVVWKLDRLGRSMKHLISLVGELRERGINFRSLTDSIDTSSPMGRFFFYVMGALAEMERELIIERTMAGLAAARNKGRIGGRPPKSGTGEKPYKCPECGKSFSTTGNLTVHQRTHTGEKPYKCPECGKSFSDPGALVRHQRTHTGEKPYKCPECGKSFSQSSNLVRHQRTHTGEKPYKCPECGKSFSRSDHLTNHQRTHTGKKTSGQAGQ

SEQ ID NO: 68 - protein, 267 aa, Artificial Sequence
  Synthetic construct
MLIGYVRVSTNDQNTDLQRNALVCAGCEQIFEDKLSGTRTDRPGLKRALKRLQKGDTLVVWKLDRLGRSMKHLISLVGELRERGINFRSLTDSIDTSSPMGRFFFYVMGALAEMERELIIERTMAGLAAARNKGRIGGRPPKSGTGEKPYKCPECGKSFSRKDNLKNHQRTHTGEKPYKCPECGKSFSRSDHLTNHQRTHTGEKPYKCPECGKSFSDPGNLVRHQRTHTGEKPYKCPECGKSFSRKDNLKNHQRTHTGKKTSGQAGQ

SEQ ID NO: 69 - protein, 267 aa, Artificial Sequence
  Synthetic construct
MLIGYVRVSTNDQNTDLQRNALVCAGCEQIFEDKLSGTRTDRPGLKRALKRLQKGDTLVVWKLDRLGRSMKHLISLVGELRERGINFRSLTDSIDTSSPMGRFFFYVMGALAEMERELILERVMAGIAAARNKGRRWGRPPKSGTGEKPYKCPECGKSFSQRANLRAHQRTHTGEKPYKCPECGKSFSQSSSLVRHQRTHTGEKPYKCPECGKSFSTTGNLTVHQRTHTGEKPYKCPECGKSFSQRAHLERHQRTHTGKKTSGQAGQ

SEQ ID NO: 70 - protein, 267 aa, Artificial Sequence
  Synthetic construct
MLIGYVRVSTNDQNTDLQRNALVCAGCEQIFEDKLSGTRTDRPGLKRALKRLQKGDTLVVWKLDRLGRSMKHLISLVGELRERGINFRSLTDSIDTSSPMGRFFFYVMGALAEMERELILERVMAGIAAARNKGRRWGRPPKSGTGEKPYKCPECGKSFSQRANLRAHQRTHTGEKPYKCPECGKSFSRRDELNVHQRTHTGEKPYKCPECGKSFSQLAHLRAHQRTHTGEKPYKCPECGKSFSQRAHLERHQRTHTGKKTSGQAGQ

SEQ ID NO: 71 - protein, 267 aa, Artificial Sequence
  Synthetic construct
MLIGYVRVSTNDQNTDLQRNALVCAGCEQIFEDKLSGTRTDRPGLKRALKRLQKGDTLVVWKLDRLGRSMKHLISLVGELRERGINFRSLTDSIDTSSPMGRFFFYVMGALAEMERELILERVMAGIAAARNKGRRWGRPPKSGTGEKPYKCPECGKSFSRRDELNVHQRTHTGEKPYKCPECGKSFSRSDHLTNHQRTHTGEKPYKCPECGKSFSQLAHLRAHQRTHTGEKPYKCPECGKSFSQRAHLERHQRTHTGKKTSGQAGQ

SEQ ID NO: 72 - protein, 267 aa, Artificial Sequence
  Synthetic construct
MLIGYVRVSTNDQNTDLQRNALVCAGCEQIFEDKLSGTRTDRPGLKRALKRLQKGDTLVVWKLDRLGRSMKHLISLVGELRERGINFRSLTDSIDTSSPMGRFFFYVMGALAEMERELIIERTMAGLAAARNKGRIGGRPPKSGTGEKPYKCPECGKSFSTSGSLVRHQRTHTGEKPYKCPECGKSFSRSDKLVRHQRTHTGEKPYKCPECGKSFSQSGDLRRHQRTHTGEKPYKCPECGKSFSTSGELVRHQRTHTGKKTSGQAGQ

SEQ ID NO: 73 - protein, 267 aa, Artificial Sequence
  Synthetic construct
MLIGYVRVSTNDQNTDLQRNALVCAGCEQIFEDKLSGTRTDRPGLKRALKRLQKGDTLVVWKLDRLGRSMKHLISLVGELRERGINFRSLTDSIDTSSPMGRFFFYVMGALAEMERELIIERTSAGRAAAINKGRIMGRPRKSGTGEKPYKCPECGKSFSQLAHLRAHQRTHTGEKPYKCPECGKSFSQLAHLRAHQRTHTGEKPYKCPECGKSFSDPGHLVRHQRTHTGEKPYKCPECGKSFSDSGNLRVHQRTHTGKKTSGQAGQ

SEQ ID NO: 74 - protein, 267 aa, Artificial Sequence
  Synthetic construct
MLIGYVRVSTNDQNTDLQRNALVCAGCEQIFEDKLSGTRTDRPGLKRALKRLQKGDTLVVWKLDRLGRSMKHLISLVGELRERGINFRSLTDSIDTSSPMGRFFFYVMGALAEMERELILERVMAGIAAARNKGRRWGRPPKSGTGEKPYKCPECGKSFSQRAHLERHQRTHTGEKPYKCPECGKSFSTTGNLTVHQRTHTGEKPYKCPECGKSFSDSGNLRVHQRTHTGEKPYKCPECGKSFSQSSNLVRHQRTHTGKKTSGQAGQ

SEQ ID NO: 75 - protein, 267 aa, Artificial Sequence
  Synthetic construct
MLIGYVRVSTNDQNTDLQRNALVCAGCEQIFEDKLSGTRTDRPGLKRALKRLQKGDTLVVWKLDRLGRSMKHLISLVGELRERGINFRSLTDSIDTSSPMGRFFFYVMGALAEMERELIIERTMAGIAAARNKGRRFGRPPKSGTGEKPYKCPECGKSFSTHLDLIRHQRTHTGEKPYKCPECGKSFSTTGNLTVHQRTHTGEKPYKCPECGKSFSQSSSLVRHQRTHTGEKPYKCPECGKSFSRSDNLVRHQRTHTGKKTSGQAGQ

SEQ ID NO: 76 - protein, 267 aa, Artificial Sequence
  Synthetic construct
MLIGYVRVSTNDQNTDLQRNALVCAGCEQIFEDKLSGTRTDRPGLKRALKRLQKGDTLVVWKLDRLGRSMKHLISLVGELRERGINFRSLTDSIDTSSPMGRFFFYVMGALAEMERELIIERTMAGIAAARNKGRRFGRPPKSGTGEKPYKCPECGKSFSRSDKLVRHQRTHTGEKPYKCPECGKSFSRRDELNVHQRTHTGEKPYKCPECGKSFSQSSSLVRHQRTHTGEKPYKCPECGKSFSRSDHLTNHQRTHTGKKTSGQAGQ

SEQ ID NO: 77 - protein, 267 aa, Artificial Sequence
  Synthetic construct
MLIGYVRVSTNDQNTDLQRNALVCAGCEQIFEDKLSGTRTDRPGLKRALKRLQKGDTLVVWKLDRLGRSMKHLISLVGELRERGINFRSLTDSIDTSSPMGRFFFYVMGALAEMERELIIERTMAGLAAARNKGRIGGRPPKSGTGEKPYKCPECGKSFSQRAHLERHQRTHTGEKPYKCPECGKSFSTSGNLVRHQRTHTGEKPYKCPECGKSFSRSDELVRHQRTHTGEKPYKCPECGKSFSHKNALQNHQRTHTGKKTSGQAGQ

SEQ ID NO: 78 - protein, 267 aa, Artificial Sequence
  Synthetic construct
MLIGYVRVSTNDQNTDLQRNALVCAGCEQIFEDKLSGTRTDRPGLKRALKRLQKGDTLVVWKLDRLGRSMKHLISLVGELRERGINFRSLTDSIDTSSPMGRFFFYVMGALAEMERELIIERTMAGLAAARNKGRIGGRPPKSGTGEKPYKCPECGKSFSRRDELNVHQRTHTGEKPYKCPECGKSFSQSSNLVRHQRTHTGEKPYKCPECGKSFSQSSSLVRHQRTHTGEKPYKCPECGKSFSTTGNLTVHQRTHTGKKTSGQAGQ

SEQ ID NO: 79 - protein, 267 aa, Artificial Sequence
  Synthetic construct
MLIGYVRVSTNDQNTDLQRNALVCAGCEQIFEDKLSGTRTDRPGLKRALKRLQKGDTLVVWKLDRLGRSMKHLISLVGELRERGINFRSLTDSIDTSSPMGRFFFYVMGALAEMERELILERVMAGIAAARNKGRRWGRPPKSGTGEKPYKCPECGKSFSTTGNLTVHQRTHTGEKPYKCPECGKSFSQSSNLVRHQRTHTGEKPYKCPECGKSFSQRAHLERHQRTHTGEKPYKCPECGKSFSQKSSLIAHQRTHTGKKTSGQAGQ

SEQ ID NO: 80 - protein, 267 aa, Artificial Sequence
  Synthetic construct
MLIGYVRVSTNDQNTDLQRNALVCAGCEQIFEDKLSGTRTDRPGLKRALKRLQKGDTLVVWKLDRLGRSMKHLISLVGELRERGINFRSLTDSIDTSSPMGRFFFYVMGALAEMERELIIERTSAGRAAAINKGRIMGRPRKSGTGEKPYKCPECGKSFSDPGALVRHQRTHTGEKPYKCPECGKSFSQSSSLVRHQRTHTGEKPYKCPECGKSFSQLAHLRAHQRTHTGEKPYKCPECGKSFSQRANLRAHQRTHTGKKTSGQAGQ

SEQ ID NO: 81 - protein, 938 aa, Artificial Sequence
  Synthetic construct
MRSPKKKRKVQVDLRTLGYSQQQQEKIKPKVRSTVAQHHEALVGHGFTHAHIVALSQHPAALGTVAVTYQHIITALPEATHEDIVGVGKQWSGARALEALLTDAGELRGPPLQLDTGQLVKIAKRGGVTAMEAVHASRNALTGAPLNLTPDQVVAIASNGGGKQALETVQRLLPVLCQDHGLTPDQVVAIASHDGGKQALETVQRLLPVLCQDHGLTPDQVVAIASNIGGKQALETVQRLLPVLCQDHGLTPDQVVAIASNGGGKQALETVQRLLPVLCQDHGLTPDQVVAIASNGGGKQALETVQRLLPVLCQDHGLTPDQVVAIASNIGGKQALETVQRLLPVLCQDHGLTPDQVVAIASHDGGKQALETVQRLLPVLCQDHGLTPDQVVAIASNIGGKQALETVQRLLPVLCQDHGLTPDQVVAIVSHDGGKQALETVQRLLPVLCQDHGLTPDQVVAIVSHDGGKQALETVQRLLPVLCQDHGLTPDQVVAIVSNGGGKQALETVQRLLPVLCQDHGLTPDQVVAIASNNGGKQALETVQRLLPVLCQDHGLTPDQVVAIASHDGGKQALETVQRLLPVLCQDHGLTPDQVVAIASNIGGKQALETVQRLLPVLCQDHGLTPDQVVAIASNNGGKQALETVQRLLPVLCQDHGLTPDQVVAIASHDGGKQALESIVAQLSRPDPALAALTNDHLVALACLGGRPAMDAVKKGLPHAPELIRRVNRRIGERTSHRVAGSQLVKSELEEKKSELRHKLKYVPHEYIELIEIARNSTQDRILEMKVMEFFMKVYGYRGKHLGGSRKPDGAIYTVGSPIDYGVIVDTKAYSGGYNLPIGQADEMQRYVEENQTRNKHINPNEWWKVYPSSVTEFKFLFVSGHFKGNYKAQLTRLNHITNCNGAVLSVEELLIGGEMIKAGTLTLEEVRRKFNNGEINF

SEQ ID NO: 82 - protein, 34 aa, Artificial Sequence
  Synthetic construct
NGNNHDNGHDNINGNGNIHDNIHDHDNGNNHDNI

SEQ ID NO: 83 - protein, 30 aa, Artificial Sequence
  Synthetic construct
HDNINNNGHDNINNNGNINGHDNININGNG

SEQ ID NO: 84 - protein, 34 aa, Artificial Sequence
  Synthetic construct
HDHDNGNNHDNINNHDNGHDNGHDNINGNGNGNG

SEQ ID NO: 85 - protein, 30 aa, Artificial Sequence
  Synthetic construct
NINGNGHDNGNGHDHDNINNNINGNGNNNI

SEQ ID NO: 86 - protein, 34 aa, Artificial Sequence
  Synthetic construct
HDNINNNININGNGNNNINGNIHDNGNNNIHDNG

SEQ ID NO: 87 - protein, 32 aa, Artificial Sequence
  Synthetic construct
NGHDNINGNGNIHDNIHDHDNGNNHDNINNHD

SEQ ID NO: 88 - protein, 36 aa, Artificial Sequence
  Synthetic construct
HDNGNGHDHDNINNNININGNGNNNINGNIHDNGNN

SEQ ID NO: 89 - DNA, 432 bp, Artificial Sequence
  Synthetic construct
atgagatctcctaagaaaaagaggaagatggtggacttgaggacactcggttattcgcaacagcaacaggagaaaatcaagcctaaggtcaggagcaccgtcgcgcaacaccacgaggcgcttgtggggcatggcttcactcatgcgcatattgtcgcgctttcacagcaccctgcggcgcttgggacggtggctgtcaaataccaagatatgattgcggccctgcccgaagccacgcacgaggcaattgtaggggtcggtaaacagtggtcgggagcgcgagcacttgaggcgctgctgactgtggcgggtgagcttagggggcctccgctccagctcgacaccgggcagctgctgaagatcgcgaagagagggggagtaacagcggtagaggcagtgcatgcatcgcgcaatgcactgacgggtgccccc

SEQ ID NO: 90 - protein, 144 aa, Artificial Sequence
  Synthetic construct
MRSPKKKRKMVDLRTLGYSQQQQEKIKPKVRSTVAQHHEALVGHGFTHAHIVALSQHPAALGTVAVKYQDMIAALPEATHEAIVGVGKQWSGARALEALLTVAGELRGPPLQLDTGQLLKIAKRGGVTAVEAVHASRNALTGAP

SEQ ID NO: 91 - DNA, 432 bp, Artificial Sequence
  Synthetic construct
atgagatctcctaagaaaaagaggaaggtgcaggtggatctacgcacgctcggctacagtcagcagcagcaagagaagatcaaaccgaaggtgcgttcgacagtggcgcagcaccacgaggcactggtgggccatgggtttacacacgcgcacatcgttgcgctcagccaacacccggcagcgttagggaccgtcgctgtcacgtatcagcacataatcacggcgttgccagaggcgacacacgaagacatcgttggcgtcggcaaatatcatggggcacgcgctctggaggccttgctcacggatgcgggggagttgagaggtccgccgttacagttggacacaggccaacttgtgaagattgcaaaacgtggcggcgtgaccgcaatggaggcagtgcatgcatcgcgcaatgcactgacgggtgccccc

SEQ ID NO: 92 - protein, 144 aa, Artificial Sequence
  Synthetic construct
MRSPKKKRKVQVDLRTLGYSQQQQEKIKPKVRSTVAQHHEALVGHGFTHAHIVALSQHPAALGTVAVTYQHIITALPEATHEDIVGVGKYHGARALEALLTDAGELRGPPLQLDTGQLVKIAKRGGVTAMEAVHASRNALTGAP

SEQ ID NO: 93 - DNA, 435 bp, Artificial Sequence
  Synthetic construct
atgagatctcctaagaaaaagaggaaggtgcaggtggatctacgcacgctcggctacagtcagcagcagcaagagaagatcaaaccgaaggtgcgttcgacagtggcgcagcaccacgaggcactggtgggccatgggtttacacacgcgcacatcgttgcgctcagccaacacccggcagcgttagggaccgtcgctgtcacgtatcagcacataatcacggcgttgccagaggcgacacacgaagacatcgttggcgtcggcaaatcgcggtcgggggcacgcgctctggaggccttgctcacggatgcgggggagttgagaggtccgccgttacagttggacacaggccaacttgtgaagattgcaaaacgtggcggcgtgaccgcaatggaggcagtgcatgcatcgcgcaatgcactgacgggtgccccc

SEQ ID NO: 94 - protein, 145 aa, Artificial Sequence
  Synthetic construct
MRSPKKKRKVQVDLRTLGYSQQQQEKIKPKVRSTVAQHHEALVGHGFTHAHIVALSQHPAALGTVAVTYQHIITALPEATHEDIVGVGKSRSGARALEALLTDAGELRGPPLQLDTGQLVKIAKRGGVTAMEAVHASRNALTGAP

SEQ ID NO: 95 - DNA, 435 bp, Artificial Sequence
  Synthetic construct
atgagatctcctaagaaaaagaggaaggtgcaggtggatctacgcacgctcggctacagtcagcagcagcaagagaagatcaaaccgaaggtgcgttcgacagtggcgcagcaccacggggcactggtgggccatgggtttacacacgcgcacatcgttgcgctcagccaacacccggcagcgttagggaccgtcgctgtcacgtatcagcacataatcacggcgttgccagaggcgacacacgaagacatcgttggcgtcggcaaacggggggctggtgcacgcgctctggaggccttgctcacggatgcgggggagttgagaggtccgccgttacagttggacacaggccaacttgtgaagattgcaaaacgtggcggcgtgaccgcaatggaggcagtgcatgcatcgcgcaatgcactgacgggtgccccc

SEQ ID NO: 96 - protein, 145 aa, Artificial Sequence
  Synthetic construct
MRSPKKKRKVQVDLRTLGYSQQQQEKIKPKVRSTVAQHHGALVGHGFTHAHIVALSQHPAALGTVAVTYQHIITALPEATHEDIVGVGKRGAGARALEALLTDAGELRGPPLQLDTGQLVKIAKRGGVTAMEAVHASRNALTGAP

SEQ ID NO: 97 - DNA, 435 bp, Artificial Sequence
  Synthetic construct
atgagatctcctaagaaaaagaggaaggtgcaggtggatctacgcacgctcggctacagtcagcagcagcaagagaagatcaaaccgaaggtgcgttcgacagtggcgcagcaccacgaggcactggtgggccatgggtttacacacgcgcacatcgttgcgctcagccaacacccggcagcgttagggaccgtcgctgtcacgtatcagcacataatcacggcgttgccagaggcgacacacgaagacatcgttggcgtcggcaaacagtggtccggcgcacgcgccctggaggccttgctcacggatgcgggggagttgagaggtccgccgttacagttggacacaggccaacttgtgaagattgcaaaacgtggcggcgtgaccgcaatggaggcagtgcatgcatcgcgcaatgcactgacgggtgccccc

SEQ ID NO: 98 - protein, 1080 aa, Artificial Sequence
  Synthetic construct
  MISC_FEATURE (498)..(498): Xaa is Q, S, R or Y
  MISC_FEATURE (499)..(499): Xaa is W, R or G
  MISC_FEATURE (500)..(500): Xaa is S, A or H
MKIEEGKLVIWINGDKGYNGLAEVGKKFEKDTGIKVTVEHPDKLEEKFPQVAATGDGPDIIFWAHDRFGGYAQSGLLAEITPDKAFQDKLYPFTWDAVRYNGKLIAYPIAVEALSLIYNKDLLPNPPKTWEEIPALDKELKAKGKSALMFNLQEPYFTWPLIAADGGYAFKYENGKYDIKDVGVDNAGAKAGLTFLVDLIKNKHMNADTDYSIAEAAFNKGETAMTINGPWAWSNIDTSKVNYGVTVLPTFKGQPSKPFVGVLSAGINAASPNKELAKEFLENYLLTDEGLEAVNKDKPLGAVALKSYEEELAKDPRIAATMENAQKGEIMPNIPQMSAFWYAVRTAVINAASGRQTVDEALKDAQTNSSSNNNNNNNNNNLGIEGRISEFGSPARPPRAKPAPRRRSAQPSDASPAAQVDLRTLGYSQQQQEKIKPKVRSTVAQHHEALVGHGFTHAHIVALSQHPAALGTVAVTYQHIITALPEATHEDIVGVGKXXXGARALEALLTDAGELLRGPPLQLDTGQLVKIAKRGGVTAMEAVHASRNALTGAPLNLTPDQVVAIASNIGGKQALETVQRLLPVLCQDHGLTPDQVVAIASNGGGKQALETVQRLLPVLCQDHGLTPDQVVAIASNIGGKQALETVQRLLPVLCQDHGLTPDQVVAIASNIGGKQALETVQRLLPVLCQDHGLTPDQVVAIASNIGGKQALETVQRLLPVLCQDHGLTPDQVVAIASHDGGKQALETVQRLLPVLCQDHGLTPDQVVAIASHDGGKQALETVQRLLPVLCQDHGLTPDQVVAIASHDGGKQALETVQRLLPVLCQDHGLTPDQVVAIVSHDGGKQALETVQRLLPVLCQDHGLTPDQVVAIVSHDGGKQALETVQRLLPVLCQDHGLTPDQVVAIVSNGGGKQALETVQRLLPVLCQDHGLTPDQVVAIASHDGGKQALETVQRLLPVLCQDHGLTPDQVVAIASHDGGKQALETVQRLLPVLCQDHGLTPDQVVAIASNIGGKQALETVQRLLPVLCQDHGLTPDQVVAIASNIGGKQALESIVAQLSRPDPALAALTNDHLVALACLG

SEQ ID NO: 99 - protein, 830 aa, Artificial Sequence
  Synthetic construct
  MISC_FEATURE (249)..(249): Xaa is Q, S, R or Y
  MISC_FEATURE (250)..(250): Xaa is W, R or G
  MISC_FEATURE (251)..(251): Xaa is S, A or H
MLIGYVRVSTNDQNTDLQRNALVCAGCEQIFEDKLSGTRTDRPGLKRALKRLQKGDTLVVWKLDRLGRSMKHLISLVGELRERGINFRSLTDSIDTSSPMGRFFFYVMGALAEMERELIIERTMAGLAAARNKGRIGGRPPKSGSPRPPRAKPAPRRRAAQPSDASPAAQVDLRTLGYSQQQQEKIKPKVRSTVAQHHEALVGHGFTHAHIVALSQHPAALGTVAVTYQHIITALPEATHEDIVGVGKXXXGARALEALLTDAGELRGPPLQLDTGQLVKIAKRGGVTAMEAVHASRNALTGAPLNLTPDQVVAIASNIGGKQALETVQRLLPVLCQDHGLTPDQVVAIASNGGGKQALETVQRLLPVLCQDHGLTPDQVVAIASNIGGKQALETVQRLLPVLCQDHGLTPDQVVAIASNIGGKQALETVQRLLPVLCQDHGLTPDQVVAIASNIGGKQALETVQRLLPVLCQDHGLTPDQVVAIASHDGGKQALETVQRLLPVLCQDHGLTPDQVVAIASHDGGKQALETVQRLLPVLCQDHGLTPDQVVAIASHDGGKQALETVQRLLPVLCQDHGLTPDQVVAIVSHDGGKQALETVQRLLPVLCQDHGLTPDQVVAIVSHDGGKQALETVQRLLPVLCQDHGLTPDQVVAIVSNGGGKQALETVQRLLPVLCQDHGLTPDQVVAIASHDGGKQALETVQRLLPVLCQDHGLTPDQVVAIASHDGGKQALETVQRLLPVLCQDHGLTPDQVVAIASNIGGKQALETVQRLLPVLCQDHGLTPDQVVAIASNIGGKQALESIVAQLSRPDPALAALTNDHLVALACLG

SEQ ID NO: 100 - protein, 839 aa, Artificial Sequence
  Synthetic construct
  MISC_FEATURE (112)..(112): Xaa is Q, S, R or Y
  MISC_FEATURE (113)..(113): Xaa is W, R or R
  MISC_FEATURE (114)..(114): Xaa is S, A or H
MAQAASGSPRPPRAKPAPRRRAAQPSDASPAAQVDLRTLGYSQQQQEKIKPKVRSTVAQHHEALVGHGFTHAHIVALSQHPAALGTVAVTYQHIITALPEATHEDIVGVGKXXXGARALEALLTDAGELRGPPLQLDTGQLVKIAKRGGVTAMEAVHASRNALTGAPLNLTPDQVVAIASNIGGKQALETVQRLLPVLCQDHGLTPDQVVAIASNGGGKQALETVQRLLPVLCQDHGLTPDQVVAIASNIGGKQALETVQRLLPVLCQDHGLTPDQVVAIASNIGGKQALETVQRLLPVLCQDHGLTPDQVVAIASNIGGKQALETVQRLLPVLCQDHGLTPDQVVAIASHDGGKQALETVQRLLPVLCQDHGLTPDQVVAIASHDGGKQALETVQRLLPVLCQDHGLTPDQVVAIASHDGGKQALETVQRLLPVLCQDHGLTPDQVVAIVSHDGGKQALETVQRLLPVLCQDHGLTPDQVVAIVSHDGGKQALETVQRLLPVLCQDHGLTPDQVVAIVSNGGGKQALETVQRLLPVLCQDHGLTPDQVVAIASHDGGKQALETVQRLLPVLCQDHGLTPDQVVAIASHDGGKQALETVQRLLPVLCQDHGLTPDQVVAIASNIGGKQALETVQRLLPVLCQDHGLTPDQVVAIASNIGGKQALESIVAQLSRPDPALAALTNDHLVALACLGGRPAMDAVKKGLPHAPELIRRVNRRIGERTSHRVADYAQVVRVLEFFQCHSHPAYAFDEAMTQFGMSGQAGQASPKKKRKVGRADALDDFDLDMLGSDALDDFDLDMLGSDALDDFDLDMLGSDALDDFDLDMLINYPYDVPDYAS

SEQ ID NO: 101 - protein, 30 aa, Artificial Sequence
  Synthetic construct
NINGNININIHDHDHDHDHDNIHDHDNINI

SEQ ID NO: 102 - protein, 33 aa, Artificial Sequence
  Synthetic construct
LTPDQLVKIAKRGGTAMEAVHASRNALTGAPLN

SEQ ID NO: 103 - protein, 4 aa, Artificial Sequence
  Synthetic construct
KRGG

SEQ ID NO: 104 - protein, 4 aa, Artificial Sequence
  Synthetic construct
LDYE

SEQ ID NO: 105 - protein, 4 aa, Artificial Sequence
  Synthetic construct
INLV

SEQ ID NO: 106 - protein, 4 aa, Artificial Sequence
  Synthetic construct
YSKK

SEQ ID NO: 107 - protein, 4 aa, Artificial Sequence
  Synthetic construct
NMAH

SEQ ID NO: 108 - protein, 4 aa, Artificial Sequence
  Synthetic construct
SPTN

SEQ ID NO: 109 - protein, 4 aa, Artificial Sequence
  Synthetic construct
SNTR

SEQ ID NO: 110 - protein, 4 aa, Artificial Sequence
  Synthetic construct
LTTT

SEQ ID NO: 111 - protein, 4 aa, Artificial Sequence
  Synthetic construct
VADL

SEQ ID NO: 112 - protein, 4 aa, Artificial Sequence
  Synthetic construct
MVLS

SEQ ID NO: 113 - protein, 4 aa, Artificial Sequence
  Synthetic construct
YNGR

SEQ ID NO: 114 - protein, 4 aa, Artificial Sequence
  Synthetic construct
RIPR

SEQ ID NO: 115 - protein, 4 aa, Artificial Sequence
  Synthetic construct
YSKI

SEQ ID NO: 116 - protein, 4 aa, Artificial Sequence
  Synthetic construct
LTQY

SEQ ID NO: 117 - protein, 4 aa, Artificial Sequence
  Synthetic construct
YLSK

SEQ ID NO: 118 - protein, 4 aa, Artificial Sequence
  Synthetic construct
LRPN

SEQ ID NO: 119 - protein, 4 aa, Artificial Sequence
  Synthetic construct
LFTN

SEQ ID NO: 120 - protein, 4 aa, Artificial Sequence
  Synthetic construct
LLTN

SEQ ID NO: 121 - protein, 4 aa, Artificial Sequence
  Synthetic construct
EEDK

SEQ ID NO: 122 - protein, 4 aa, Artificial Sequence
  Synthetic construct
VTAM

SEQ ID NO: 123 - protein, 4 aa, Artificial Sequence
  Synthetic construct
CPSR

SEQ ID NO: 124 - protein, 4 aa, Artificial Sequence
  Synthetic construct
LTRV

SEQ ID NO: 125 - protein, 4 aa, Artificial Sequence
  Synthetic construct
KGDL

SEQ ID NO: 126 - protein, 4 aa, Artificial Sequence
  Synthetic construct
QKAL

SEQ ID NO: 127 - protein, 4 aa, Artificial Sequence
  Synthetic construct
LYLL

SEQ ID NO: 128 - protein, 4 aa, Artificial Sequence
  Synthetic construct
WISV

SEQ ID NO: 129 - protein, 4 aa, Artificial Sequence
  Synthetic construct
GDQV

SEQ ID NO: 130 - protein, 4 aa, Artificial Sequence
  Synthetic construct
CPSR

SEQ ID NO: 131 - protein, 145 aa, Artificial Sequence
  Synthetic construct
  misc_feature (89)..(93): Xaa can be any naturally occurring amino acid
MRSPKKKRKVQVDLRTLGYSQQQQEKIKPKVRSTVAQHHEALVGHGFTHAHIVALSQHPAALGTVAVTYQHIITALPEATHEDIVGVGXXXXXARALEALLTDAGELRGPPLQLDTGQLVKIAKRGGVTAMEAVHASRNALTGAP

SEQ ID NO: 132 - protein, 5 aa, Artificial Sequence
  Synthetic construct
KRPAG

SEQ ID NO: 133 - protein, 5 aa, Artificial Sequence
  Synthetic construct
KRPSG

SEQ ID NO: 134 - protein, 32 aa, Artificial Sequence
  Synthetic construct
LTPDVVAISNNGGKQALETVQRLLPVLCQDGH

SEQ ID NO: 135 - protein, 4 aa, Artificial Sequence
  Synthetic construct
SNNG

SEQ ID NO: 136 - protein, 4 aa, Artificial Sequence
  Synthetic construct
RGGG

SEQ ID NO: 137 - protein, 4 aa, Artificial Sequence
  Synthetic construct
RGGR

SEQ ID NO: 138 - protein, 4 aa, Artificial Sequence
  Synthetic construct
RGVR

SEQ ID NO: 139 - protein, 4 aa, Artificial Sequence
  Synthetic construct
KGGG

SEQ ID NO: 140 - protein, 4 aa, Artificial Sequence
  Synthetic construct
SGGG

SEQ ID NO: 141 - protein, 4 aa, Artificial Sequence
  Synthetic construct
GGRG

SEQ ID NO: 142 - protein, 4 aa, Artificial Sequence
  Synthetic construct
LGGS

SEQ ID NO: 143 - protein, 4 aa, Artificial Sequence
  Synthetic construct
MDNI

SEQ ID NO: 144 - protein, 4 aa, Artificial Sequence
  Synthetic construct
RVMA

SEQ ID NO: 145 - protein, 4 aa, Artificial Sequence
  Synthetic construct
LASV

SEQ ID NO: 146 - protein, 4 aa, Artificial Sequence
  Synthetic construct
VGTG

SEQ ID NO: 147 - protein, 4 aa, Artificial Sequence
  Synthetic construct
QGGG

SEQ ID NO: 148 - DNA, 118 bp, Artificial Sequence
  Primer
ttaattaagagtctagaaatataaaccccctccaaccaggtgctaactgtaaaccatggttttggattagcacctggttggagggggtttataagatctaggaggaatttaaaatgag

SEQ ID NO: 149 - DNA, 117 bp, Artificial Sequence
  Primer
actgacctagagaagcttatataaaccccctccaaccaggtgctaatccaaaaccatggtttacagttagcacctggttggagggggtttatactgcagttatttgtacagttcatc

SEQ ID NO: 150 - DNA, 116 bp, Artificial Sequence
  Primer
ttaattaagagtctagattagcacctggttggagggggtttataaggttttggtaccaaatgtctataaaccccctccaaccaggtgctaaagatctaggaggaatttaaaatgag

SEQ ID NO: 151 - DNA, 116 bp, Artificial Sequence; identical to SEQ ID NO: 150
  Primer

SEQ ID NO: 152 - DNA, 116 bp, Artificial Sequence
  Primer
actgacctagagaagcttttagcacctggttggagggggtttatagacatttggtaccaaaaccttataaaccccctccaaccaggtgctaactgcagttatttgtacagttcatc

SEQ ID NO: 153 - DNA, 116 bp, Artificial Sequence
  Primer
ttaattaagagtctagattagcacctggttggagggggtttatatccaaaaccatggtttacagtataaaccccctccaaccaggtgctaaagatctaggaggaatttaaaatgag

SEQ ID NO: 154 - DNA, 116 bp, Artificial Sequence
  Primer
actgacctagagaagcttttagcacctggttggagggggtttatatccaaaaccatggtttacagtataaaccccctccaaccaggtgctaactgcagttatttgtacagttcatc

SEQ ID NO: 155 - DNA, 122 bp, Artificial Sequence
  Primer
ttaattaagagtctagattagcacctggttggagggggtttatagcttccaaaaccatggtttacagggttataaaccccctccaaccaggtgctaaagatctaggaggaatttaaaatgag

SEQ ID NO: 156 - DNA, 128 bp, Artificial Sequence
  Primer
ttaattaagagtctagattagcacctggttggagggggtttatagcttcatccaaaaccatggtttacagggttcctataaaccccctccaaccaggtgctaaagatctaggaggaatttaaaatgag

SEQ ID NO: 157 - DNA, 128 bp, Artificial Sequence
  Primer
actgacctagagaagcttttagcacctggttggagggggtttatagcaaccctgtaaaccatggttttggatgaagctataaaccccctccaaccaggtgctaactgcagttatttgtacagttcatc

SEQ ID NO: 158 - DNA, 140 bp, Artificial Sequence
  Primer
ttaattaagagtctagattagcacctggttggagggggtttatagcttcagcttcatccaaaaccatggtttacagggttccggttcctataaaccccctccaaccaggtgctaaagatctaggaggaatttaaaatgag

SEQ ID NO: 159 - DNA, 140 bp, Artificial Sequence; identical to SEQ ID NO: 158
  Primer

SEQ ID NO: 160 - DNA, 110 bp, Artificial Sequence
  Primer
ttaattaagagtctagattagcacctggttggagggggtttataaaaaccatggtttatataaaccccctccaaccaggtgctaaagatctaggaggaatttaaaatgag

SEQ ID NO: 161 - DNA, 110 bp, Artificial Sequence
  Primer
actgacctagagaagcttttagcacctggttggagggggtttatataaaccatggtttttataaaccccctccaaccaggtgctaactgcagttatttgtacagttcatc

SEQ ID NO: 162 - DNA, 116 bp, Artificial Sequence
  Primer
ttaattaagagtctagattagcacctggttggagggggtttatatccaaaaccggggtttacagtataaaccccctccaaccaggtgctaaagatctaggaggaatttaaaatgag

SEQ ID NO: 163 - DNA, 116 bp, Artificial Sequence
  Primer
actgacctagagaagcttttagcacctggttggagggggtttatactgtaaaccccggttttggatataaaccccctccaaccaggtgctaactgcagttatttgtacagttcatc

SEQ ID NO: 164 - DNA, 116 bp, Artificial Sequence
  Primer
ttaattaagagtctagattagcacctggttggagggggtttatacgaaatattataaattatcatataaaccccctccaaccaggtgctaaagatctaggaggaatttaaaatgag

SEQ ID NO: 165 - DNA, 116 bp, Artificial Sequence
  Primer
actgacctagagaagcttttagcacctggttggagggggtttatatgataatttataatatttcgtataaaccccctccaaccaggtgctaactgcagttatttgtacagttcatc

SEQ ID NO: 166 - DNA, 128 bp, Artificial Sequence
  Primer
ttaattaagagtctagattagcacctggttggagggggtttatagcttcatccaaaaccggggtttacagggttcctataaaccccctccaaccaggtgctaaagatctaggaggaatttaaaatgag

SEQ ID NO: 167 - DNA, 128 bp, Artificial Sequence
  Primer
actgacctagagaagcttttagcacctggttggagggggtttatagcaaccctgtaaaccggggttttggatgaagctataaaccccctccaaccaggtgctaactgcagttatttgtacagttcatc

SEQ ID NO: 168 - DNA, 128 bp, Artificial Sequence
  Primer
ttaattaagagtctagattagcacctggttggagggggtttatagcttcacgaaatattataaattatcaggttcctataaaccccctccaaccaggtgctaaagatctaggaggaatttaaaatgag

SEQ ID NO: 169 - DNA, 128 bp, Artificial Sequence
  Primer
actgacctagagaagcttttagcacctggttggagggggtttatagcaacctgataatttataatatttcgtgaagctataaaccccctccaaccaggtgctaactgcagttatttgtacagttcatc

SEQ ID NO: 170 - DNA, 128 bp, Artificial Sequence
  Primer
ttaattaagagagatctttagcacctggttggagggggtttatagcttcatccaaaaccatggtttacagggttcctataaaccccctccaaccaggtgctaagcgatctgcatctcaattagtcagc

SEQ ID NO: 171 - DNA, 128 bp, Artificial Sequence
  Primer
actgacctagagaagcttttagcacctggttggagggggtttatagcaaccctgtaaaccatggttttggatgaagctataaaccccctccaaccaggtgctaatttgcaaaagcctaggcctccaaa

SEQ ID NO: 172 - DNA, 107 bp, Artificial Sequence
  Primer
ttaattaagagagatctgcgggaggcgtgtccaaaaccatggtttacagggttcctataaaccccctccaaccaggtgctaagcgatctgcatctcaattagtcagc

SEQ ID NO: 173 - DNA, 107 bp, Artificial Sequence
  Primer
actgacctagagaagcttttagcacctggttggagggggtttatagcaaccctgtaaaccatggttttggacacgcctcccgctttgcaaaagcctaggcctccaaa

SEQ ID NO: 174 - DNA, 140 bp, Artificial Sequence
  Primer
ttaattaagagagatctttagcacctggttggagggggtttatagcttcagcttcatccaaaaccatggtttacagggttccggttcctataaaccccctccaaccaggtgctaagcgatctgcatctcaattagtcagc

SEQ ID NO: 175 - DNA, 140 bp, Artificial Sequence
  Primer
actgacctagagaagcttttagcacctggttggagggggtttatagcaaccgcaaccctgtaaaccatggttttggatgaagctgaagctataaaccccctccaaccaggtgctaatttgcaaaagcctaggcctccaaa

SEQ ID NO: 176 - DNA, 52 bp, Artificial Sequence
  Primer
agtcagtcgagagctcatggatcccggctctatgctgattggctatgtaagg

SEQ ID NO: 177 - DNA, 39 bp, Artificial Sequence
  Primer
atgctgatatctagactatcccgatttaggtgggcgacc

SEQ ID NO: 178 - DNA, 37 bp, Artificial Sequence
  Primer
agtcagtcgagagctcatgctgattggctatgtaagg

SEQ ID NO: 179 - DNA, 32 bp, Artificial Sequence
  Primer
tctagactacggatccaccgatttacgcgggc

SEQ ID NO: 180 - DNA, 39 bp, Artificial Sequence
  Primer
atcgcgtatctagactagccgaggcaggccaaggcgacg

SEQ ID NO: 181 - DNA, 39 bp, Artificial Sequence
  Primer
atcgcgtatctagactagctcatctcgaactgcgtcatg

SEQ ID NO: 182 - DNA, 43 bp, Artificial Sequence
  Primer
gtcgcccgcgtaaatcgggatccactgcagatcgggggggggc

SEQ ID NO: 183 - DNA, 43 bp, Artificial Sequence
  Primer
gtcgcccgcgtaaatcgggatccccctcgcctgcgttctcggc

SEQ ID NO: 184 - DNA, 43 bp, Artificial Sequence
  Primer
gtcgcccgcgtaaatcgggatccgattcgatgcctgccgtcgg

SEQ ID NO: 185 - DNA, 45 bp, Artificial Sequence
  Primer
gtcgcccgcgtaaatcgggatccaccgtgcgtgtcgctgtcactg

SEQ ID NO: 186 - DNA, 44 bp, Artificial Sequence
  Primer
gtcgcccgcgtaaatcgggatccgtggatctacgcacgctcggc

SEQ ID NO: 187 - DNA, 43 bp, Artificial Sequence
  Primer
gtcgcccgcgtaaatcgggatccacacacgcgcacatcgttgc

SEQ ID NO: 188 - DNA, 45 bp, Artificial Sequence
  Primer
gtcgcccgcgtaaatcgggatcccacgaagacatcgttggcgtcg

SEQ ID NO: 189 - DNA, 44 bp, Artificial Sequence
  Primer
gtcgcccgcgtaaatcgggatccagcgctctggaggccttgctc

SEQ ID NO: 190 - DNA, 44 bp, Artificial Sequence
  Primer
gtcgcccgcgtaaatcgggatccttggacacaggccaacttctc

SEQ ID NO: 191 - DNA, 43 bp, Artificial Sequence
  Primer
gtcgcccgcgtaaatcgggatccagcggcgtgaccgcagtgga

SEQ ID NO: 192 - DNA, 20 bp, Artificial Sequence
  Primer
ggatcccgatttacgcgggc

SEQ ID NO: 193 - DNA, 41 bp, Artificial Sequence
  Primer
atcgtagcagctagcgccaccatgctgattggctatgtaag

SEQ ID NO: 194 - DNA, 26 bp, Artificial Sequence
  Primer
ggatccagaccccgatttacgcgggc

SEQ ID NO: 195 - DNA, 74 bp, Artificial Sequence
  Synthetic construct
ttagcacctggttggagggggtttatatccaaaaccatggtttacagtataaaccccctccaaccaggtgctaa

SEQ ID NO: 196 - DNA, 74 bp, Artificial Sequence
  Synthetic construct
ttagcacctggttggagggggtttataaggttttggtaccaaatgtctataaaccccctccaaccaggtgctaa

SEQ ID NO: 197 - DNA, 74 bp, Artificial Sequence
  Synthetic construct
tataaaccccctccaaccaggtgctaactgtaaaccatggttttggattagcacctggttggagggggtttata

SEQ ID NO: 198 - DNA, 68 bp, Artificial Sequence
  Synthetic construct
ttagcacctggttggagggggtttataaaaaccatggtttatataaaccccctccaaccaggtgctaa

SEQ ID NO: 199 - DNA, 80 bp, Artificial Sequence
  Synthetic construct
ttagcacctggttggagggggtttatagcttccaaaaccatggtttacagggttataaaccccctccaaccaggtgctaa

SEQ ID NO: 200 - DNA, 86 bp, Artificial Sequence
  Synthetic construct
ttagcacctggttggagggggtttatagcttcatccaaaaccatggtttacagggttcctataaaccccctccaaccaggtgctaa

SEQ ID NO: 201 - DNA, 98 bp, Artificial Sequence
  Synthetic construct
ttagcacctggttggagggggtttatagcttcagcttcatccaaaaccatggtttacagggttccggttcctataaaccccctccaaccaggtgctaa

SEQ ID NO: 202 - DNA, 74 bp, Artificial Sequence
  Synthetic construct
ttagcacctggttggagggggtttatatccaaaaccggggtttacagtataaaccccctccaaccaggtgctaa

SEQ ID NO: 203 - DNA, 74 bp, Artificial Sequence
  Synthetic construct
ttagcacctggttggagggggtttatacgaaatattataaattatcatataaaccccctccaaccaggtgctaa

SEQ ID NO: 204 - DNA, 86 bp, Artificial Sequence
  Synthetic construct
ttagcacctggttggagggggtttatagcttcatccaaaaccggggtttacagggttcctataaaccccctccaaccaggtgctaa

SEQ ID NO: 205 - DNA, 86 bp, Artificial Sequence
  Synthetic construct
ttagcacctggttggagggggtttatagcttcacgaaatattataaattatcaggttcctataaaccccctccaaccaggtgctaa

SEQ ID NO: 206 - DNA, 65 bp, Artificial Sequence
  Synthetic construct
gcgggaggcgtgtccaaaaccatggtttacagggttcctataaaccccctccaaccaggtgctaa

SEQ ID NO: 207 - DNA, 70 bp, Artificial Sequence
  Synthetic construct
gtggtgtacagtagggggagatgcatccaaaaccatggtttacagtgcatctccccctactgtacaccac

SEQ ID NO: 208 - DNA, 82 bp, Artificial Sequence
  Synthetic construct
gtggtgtacagtagggggagatgcagctgcttccaaaaccatggtttacagggtggttgcatctccccctactgtacaccac

SEQ ID NO: 209 - protein, 4 aa, Artificial Sequence
  Synthetic construct
QWSG

SEQ ID NO: 210 - protein, 4 aa, Artificial Sequence
  Synthetic construct
RSNG

SEQ ID NO: 211 - protein, 4 aa, Artificial Sequence
  Synthetic construct
SRSG

SEQ ID NO: 212 - protein, 4 aa, Artificial Sequence
  Synthetic construct
QWSG

SEQ ID NO: 213 - DNA, 16 bp, Artificial Sequence
  Synthetic construct
gataaaccccctccaa

SEQ ID NO: 214 - DNA, 15 bp, Artificial Sequence
  Synthetic construct
ataaaccccctccaa

SEQ ID NO: 215 - protein, 35 aa, Artificial Sequence
  Synthetic construct
ATHEDIVGVGKQWSGARALEALLTDAGELRGPPLQ

SEQ ID NO: 216 - protein, 35 aa, Artificial Sequence; identical to SEQ ID NO: 215
  Synthetic construct

SEQ ID NO: 217 - protein, 5 aa, Artificial Sequence
  Synthetic construct
KQWSG

SEQ ID NO: 218 - protein, 5 aa, Artificial Sequence
  Synthetic construct
KRSNG

SEQ ID NO: 219 - protein, 5 aa, Artificial Sequence
  Synthetic construct
KSRSG

SEQ ID NO: 220 - protein, 35 aa, Artificial Sequence; identical to SEQ ID NO: 215
  Synthetic construct

SEQ ID NO: 221 - protein, 5 aa, Artificial Sequence
  Synthetic construct
KQWSG

SEQ ID NO: 222 - DNA, 16 bp, Artificial Sequence
  Synthetic construct
aataaaccccctccaa

SEQ ID NO: 223 - DNA, 16 bp, Artificial Sequence
  Synthetic construct
tataaaccccctccaa

SEQ ID NO: 224 - protein, 4 aa, Artificial Sequence
  Synthetic construct
KRGG

SEQ ID NO: 225 - protein, 34 aa, Artificial Sequence
  Synthetic construct
LTPDQVVAIASHDGGKQALETVQRLLPVLCQDHG

SEQ ID NO: 226 - protein, 4 aa, Artificial Sequence
  Synthetic construct
SHDG

SEQ ID NO: 227 - protein, 6 aa, Artificial Sequence
  Synthetic construct
ASHDGG

SEQ ID NO: 228 - DNA, 81 bp, Artificial Sequence
  Primer
  misc_feature (50)..(51): n is a, c, g, or t
  misc_feature (53)..(54): n is a, c, g, or t
tctcaactcccccgcctccgtgagcaaggcctccagagcgcgtgccccmnnmnntttgccgacgccaacgatgtcttcgtg

SEQ ID NO: 229 - DNA, 84 bp, Artificial Sequence
  Primer
  misc_feature (47)..(48): n is a, c, g, or t
  misc_feature (50)..(51): n is a, c, g, or t
  misc_feature (53)..(54): n is a, c, g, or t
  misc_feature (56)..(57): n is a, c, g, or t
tctcaactcccccgcctccgtgagcaaggcctccagagcgcgtgcmnnmnnmnnmnntttgccgacgccaacgatgtcttcgtg

SEQ ID NO: 230 - DNA, 80 bp, Artificial Sequence
  Primer
  misc_feature (43)..(44): n is a, c, g, or t
  misc_feature (46)..(47): n is a, c, g, or t
  misc_feature (49)..(50): n is a, c, g, or t
cccgcctccgtgagcaaggcctccagggcgcgtgcgccggamnnmnnmnngccgacgccaacgatgtcttcgtgtgtcgc

SEQ ID NO: 231 - DNA, 90 bp, Artificial Sequence
  Primer
  misc_feature (53)..(54): n is a, c, g, or t
  misc_feature (56)..(57): n is a, c, g, or t
  misc_feature (59)..(60): n is a, c, g, or t
  misc_feature (62)..(63): n is a, c, g, or t
ggcacccgtcagtgcattgcgccatgcatgcactgcctccactgcggtcacmnnmnnmnnmnntgcaatcttgagaagttggcctgtgtc

SEQ ID NO: 232 - DNA, 71 bp, Artificial Sequence
  Primer
agagagagaagaaaatgagatctcctaagaaaaagaggaaggtgcaggtggatctacgcacgctcggctac

SEQ ID NO: 233 - DNA, 71 bp, Artificial Sequence
  Primer
aggaagaagagaagcatgagatctcctaagaaaaagaggaaggtgatggtggacttgaggacactcggtta

SEQ ID NO: 234 - DNA, 44 bp, Artificial Sequence
  Primer
aagagaagaagaagaagcattgcgccatgcatgcactgcctcta

SEQ ID NO: 235 - DNA, 17 bp, Artificial Sequence
  Primer
cccgccacccaccgtgc

SEQ ID NO: 236 - DNA, 23 bp, Artificial Sequence
  Primer
tgctctatgcatgcactgcctcc

SEQ ID NO: 237 - DNA, 68 bp, Artificial Sequence
  Primer
agagaagagaagagaaggcgcccgcggcccaggcggcctcgggatcccctcggcctccgcgcgccaag

SEQ ID NO: 238 - DNA, 65 bp, Artificial Sequence
  Primer
agagagagagagagagtctagaggccggcctggccgctcatcccgaactgcgtcatggcctcatc

SEQ ID NO: 239 - DNA, 27 bp, Artificial Sequence
  Primer
gccccagatcctggtacgctctagagg

SEQ ID NO: 240 - DNA, 70 bp, Artificial Sequence
  Primer
atcttagcacctggttggagggggtttattgggttttcccaataaaccccctccaaccaggtgctaagat

SEQ ID NO: 241 - DNA, 70 bp, Artificial Sequence
  Primer
atcttagcacctggttggagggggtttatagggttttccctataaaccccctccaaccaggtgctaagat

SEQ ID NO: 242 - DNA, 70 bp, Artificial Sequence
  Primer
atcttagcacctggttggagggggtttatcgggttttcccgataaaccccctccaaccaggtgctaagat

SEQ ID NO: 243 - DNA, 70 bp, Artificial Sequence
  Primer
atcttagcacctggttggagggggtttatggggttttccccataaaccccctccaaccaggtgctaagat

SEQ ID NO: 244 - DNA, 20 bp, Artificial Sequence
  Primer
ttaaaagccaggacggtcac

SEQ ID NO: 245 - DNA, 20 bp, Artificial Sequence
  Primer
tgtagggagcccagaagaga

SEQ ID NO: 246 - DNA, 22 bp, Artificial Sequence
  Primer
acagtttgcattcatggagggc

SEQ ID NO: 247 - DNA, 20 bp, Artificial Sequence
  Primer
ccgagcgagcaagctcagtt

SEQ ID NO: 248 - DNA, 27 bp, Artificial Sequence
  Primer
cgcggatccccgcccagtgggactttg

SEQ ID NO: 249 - DNA, 27 bp, Artificial Sequence
  Primer
ccggaattcacctgttagagctactgc

SEQ ID NO: 250 - DNA, 54 bp, Artificial Sequence
  Primer
agagagagagagaggcggccgccctaccagggatttcagtcgatgtacacgttc

SEQ ID NO: 251 - DNA, 58 bp, Artificial Sequence
  Primer
aagaagaagaaggaagagaagtaggcctgtcatcgtcgggaagacctgcgacacctgc

SEQ ID NO: 252 - DNA, 138 bp, Artificial Sequence
  Primer
actgctatccgagtataaaccccctccaaccaggtataaaccccctccaaccaggtataaaccccctccaaccaggtataaaccccctccaaccaggtataaaccccctccaaccaggatctgcgatctaagtaagct

SEQ ID NO: 253 - DNA, 128 bp, Artificial Sequence
  Primer
ttaattaagagtctagattagcacctggttggagggggtttattgcttcatccaaaaccatggtttacagggttccaataaaccccctccaaccaggtgctaaagatctaggaggaatttaaaatgag

SEQ ID NO: 254 - DNA, 128 bp, Artificial Sequence
  Primer
actgacctagagaagcttttagcacctggttggagggggtttattgcaaccctgtaaaccatggttttggatgaagcaataaaccccctccaaccaggtgctaactgcagttatttgtacagttcatc

SEQ ID NO: 255 - DNA, 128 bp, Artificial Sequence
  Primer
ttaattaagagtctagattagcacctggttggagggggtttatcgcttcatccaaaaccatggtttacagggttccgataaaccccctccaaccaggtgctaaagatctaggaggaatttaaaatgag

SEQ ID NO: 256 - DNA, 128 bp, Artificial Sequence
  Primer
actgacctagagaagcttttagcacctggttggagggggtttatcgcaaccctgtaaaccatggttttggatgaagcgataaaccccctccaaccaggtgctaactgcagttatttgtacagttcatc

SEQ ID NO: 257 - DNA, 128 bp, Artificial Sequence
  Primer
ttaattaagagtctagattagcacctggttggagggggtttatggcttcatccaaaaccatggtttacagggttcccataaaccccctccaaccaggtgctaaagatctaggaggaatttaaaatgag

SEQ ID NO: 258 - DNA, 128 bp, Artificial Sequence
  Primer
actgacctagagaagcttttagcacctggttggagggggtttatggcaaccctgtaaaccatggttttggatgaagccataaaccccctccaaccaggtgctaactgcagttatttgtacagttcatc

SEQ ID NO: 259 - DNA, 144 bp, Artificial Sequence
  Primer
actgctatctcgagctataaaccccctccaaccaggctataaaccccctccaaccaggctataaaccccctccaaccaggctataaaccccctccaaccaggctataaaccccctccaaccaggatctgcgatctaagtaagct

SEQ ID NO: 260 - DNA, 144 bp, Artificial Sequence
  Primer
actgctatctcgagcaataaaccccctccaaccaggcaataaaccccctccaaccaggcaataaaccccctccaaccaggcaataaaccccctccaaccaggcaataaaccccctccaaccaggatctgcgatctaagtaagct

SEQ ID NO: 261 - DNA, 144 bp, Artificial Sequence
  Primer
actgctatctcgagccataaaccccctccaaccaggccataaaccccctccaaccaggccataaaccccctccaaccaggccataaaccccctccaaccaggccataaaccccctccaaccaggatctgcgatctaagtaagct

SEQ ID NO: 262 - DNA, 144 bp, Artificial Sequence
  Primer
actgctatctcgagcgataaaccccctccaaccaggcgataaaccccctccaaccaggcgataaaccccctccaaccaggcgataaaccccctccaaccaggcgataaaccccctccaaccaggatctgcgatctaagtaagct

SEQ ID NO: 263 - DNA, 25 bp, Artificial Sequence
  Primer
tcagaaacagctcttcttcaaatct

SEQ ID NO: 264 - DNA, 80 bp, Artificial Sequence
  Primer
ttaattaagagtctagaggaggcgtgtccaaaaccatggtttacagcacgcctccagatctaggaggaatttaaaatgag

SEQ ID NO: 265 - DNA, 80 bp, Artificial Sequence
  Primer
actgacctagagaagcttggaggcgtgctgtaaaccatggttttggacacgcctccctgcagttatttgtacagttcatc

SEQ ID NO: 266 - DNA, 86 bp, Artificial Sequence
  Primer
ttaattaagagagatctgctgatgcagatacagaaaccaaggttttcttacttgctgctgcgcgatctgcatctcaattagtcagc

SEQ ID NO: 267 - DNA, 82 bp, Artificial Sequence
  Primer
caccaccacggatccgcagcagcaagtaagaaaaccttggtttctgtatctgcatcagcaatttcgataagccagtaagcag

SEQ ID NO: 268 - DNA, 65 bp, Artificial Sequence
  Primer
caccaccacgcgcgcaagcttagatctggcccaggcggccaccatgctgattggctatgtaaggg

SEQ ID NO: 269 - DNA, 35 bp, Artificial Sequence
  Primer
caccaccacaccggttcccgatttaggtgggcgac

SEQ ID NO: 270 - DNA, 21 bp, Artificial Sequence
  Primer
gttcctgccaggatccactag

SEQ ID NO: 271 - DNA, 21 bp, Artificial Sequence
  Primer
gcatgtgtccagatgcatagg

SEQ ID NO: 272 - DNA, 20 bp, Artificial Sequence
  Primer
caccttctcccaggataagg

SEQ ID NO: 273 - DNA, 20 bp, Artificial Sequence
  Primer
gttggcctgtattcctctgg

SEQ ID NO: 274 - DNA, 22 bp, Artificial Sequence
  Primer
aatgaagttcccttggcacttc

SEQ ID NO: 275 - DNA, 23 bp, Artificial Sequence
  Primer
ctgaagggttttaagtgcagaag

SEQ ID NO: 276 - DNA, 22 bp, Artificial Sequence
  Primer
tgacgtcaatgacggtaaatgg

SEQ ID NO: 277 - DNA, 122 bp, Artificial Sequence
  Primer
actgacctagagaagcttttagcacctggttggagggggtttataaccctgtaaaccatggttttggaagctataaaccccctccaaccaggtgctaactgcagttatttgtacagttcatc

SEQ ID NO: 278 - DNA, 140 bp, Artificial Sequence
  Primer
actgacctagagaagcttttagcacctggttggagggggtttatagcaaccgcaaccctgtaaaccatggttttggatgaagctgaagctataaaccccctccaaccaggtgctaactgcagttatttgtacagttcatc

SEQ ID NO: 279 - DNA, 12 bp, Artificial Sequence
  Synthetic construct
gcgggaggcgtg

SEQ ID NO: 280 - DNA, 17 bp, Artificial Sequence
  Synthetic construct
tcttcattacacctgca

SEQ ID NO: 281 - DNA, 15 bp, Artificial Sequence
  Synthetic construct
cagtcagtatcaatt

SEQ ID NO: 282 - DNA, 17 bp, Artificial Sequence
  Synthetic construct
cctgcagctctcatttt

SEQ ID NO: 283 - DNA, 16 bp, Artificial Sequence
  Synthetic construct
attcttccagaattga

SEQ ID NO: 284 - DNA, 17 bp, Artificial Sequence
  Synthetic construct
cagaattgatactgact

SEQ ID NO: 285 - DNA, 16 bp, Artificial Sequence
  Synthetic construct
tcattacacctgcagc

SEQ ID NO: 286 - DNA, 18 bp, Artificial Sequence
  Synthetic construct
cttccagaattgatactg

SEQ ID NO: 287 - DNA, 15 bp, Artificial Sequence
  Synthetic construct
ataaaccccctccaa

SEQ ID NO: 288 - DNA, 74 bp, Artificial Sequence; identical to SEQ ID NO: 195
  Synthetic construct

SEQ ID NO: 289 - DNA, 74 bp, Artificial Sequence; identical to SEQ ID NO: 196
  Synthetic construct

SEQ ID NO: 290 - DNA, 74 bp, Artificial Sequence; identical to SEQ ID NO: 197
  Synthetic construct

SEQ ID NO: 291 - protein, 6 aa, Artificial Sequence
  Synthetic construct
  misc_feature (2)..(3): Xaa can be any naturally occurring amino acid
KXXGAR

SEQ ID NO: 292 - DNA, 83 bp, Artificial Sequence
  Synthetic construct
tggaaattcttccagaattgatactgactgtatggaaaatgagagctgcaggtgtaatgaagaccttctttttgagatctggt

SEQ ID NO: 293 - DNA, 77 bp, Artificial Sequence
  Synthetic construct
tggaaattcttccataattgatattgactgtatggaaggctgcgggtgtaatgaataccttctttttgagatctggt

SEQ ID NO: 294 - DNA, 77 bp, Artificial Sequence
  Synthetic construct
tggaaattcttccagaattgatactgactgtatggaaaactgcaggtgtaatgaagaccttctttttgagatctggt

SEQ ID NO: 295 - DNA, 77 bp, Artificial Sequence
  Synthetic construct
tggaaattcttccagaattgatactgactgtatggaaagctgcaggtgtaatgaagaccttctttttgagatctggt

SEQ ID NO: 296 - DNA, 76 bp, Artificial Sequence
  Synthetic construct
tggaaattcttccagaattgatactgactgtatggaagctgcaggtgtaatgaagaccttctttttgagatctggt

SEQ ID NO: 297 - DNA, 73 bp, Artificial Sequence
  Synthetic construct
tggaaattcttccagaattgatactgactgtagagctgcaggtgtaatgaagaccttctttttgagatctggt

SEQ ID NO: 298 - DNA, 72 bp, Artificial Sequence
  Synthetic construct
tggaaattcttccagaattgatactgactgtatgctgcaggtgtaatgaagaccttctttttgagatctggt

SEQ ID NO: 299 - DNA, 70 bp, Artificial Sequence
  Synthetic construct
tggaaattcttccagaattgatactgactgtgctgcaggtgtaatgaagaccttctttttgagatctggt

SEQ ID NO: 300 - DNA, 83 bp, Artificial Sequence; identical to SEQ ID NO: 292
  Synthetic construct

SEQ ID NO: 301 - DNA, 79 bp, Artificial Sequence
  Synthetic construct
tggaaattcttccagaattgatactgactgtatggaaagagctgcaggtgtaatgaagaccttctttttgagatctggt

SEQ ID NO: 302 - DNA, 78 bp, Artificial Sequence
  Synthetic construct
tggaaattcttccagaattgatactgactgtatggaagagctgcaggtgtaatgaagaccttctttttgagatctggt

SEQ ID NO: 303 - DNA, 77 bp, Artificial Sequence
  Synthetic construct
tggaaattcttccagaattgatactgactgtatggagagctgcaggtgtaatgaagaccttctttttgagatctggt

SEQ ID NO: 304 - DNA, 74 bp, Artificial Sequence
  Synthetic construct
tggaaattcttccagaattgatactgactatgagagctgcaggtgtaatgaagaccttctttttgagatctggt

SEQ ID NO: 305 - DNA, 73 bp, Artificial Sequence; identical to SEQ ID NO: 297
  Synthetic construct

SEQ ID NO: 306 - DNA, 72 bp, Artificial Sequence
  Synthetic construct
tggaaattcttccagaattgatactgactgagagctgcaggtgtaatgaagaccttctttttgagatctggt

SEQ ID NO: 307 - DNA, 72 bp, Artificial Sequence
  Synthetic construct
tggaaattcttccaggattgatactgactgagagctgcaggtgtaatgaagaccttctttttgagatctggt

SEQ ID NO: 308 - DNA, 72 bp, Artificial Sequence; identical to SEQ ID NO: 306
  Synthetic construct

SEQ ID NO: 309 - DNA, 72 bp, Artificial Sequence
  Synthetic construct
tggaaattcttccagaattgatactgactaggagctgcaggtgtaatgaagaccttctttttgagatctggt

SEQ ID NO: 310 - DNA, 83 bp, Artificial Sequence; identical to SEQ ID NO: 292
  Synthetic construct

SEQ ID NO: 311 - DNA, 81 bp, Artificial Sequence
  Synthetic construct
tggaaattcttccagaattgatactgactatggaaaatgagagctgcaggtgtaatgaagaccttctttttgagatctggt

SEQ ID NO: 312 - DNA, 80 bp, Artificial Sequence
  Synthetic construct
tggaaattcttcctcaattgatactgatatggaaaatgagagctgcaggtgtaatgaagaccttctttttgagatctggt

SEQ ID NO: 313 - DNA, 74 bp, Artificial Sequence
  Synthetic construct
tggaaattcttccagaattgatatggaaaatgagagctgcaggtgtaatgaagaccttctttttgagatctggt

SEQ ID NO: 314 - DNA, 83 bp, Artificial Sequence; identical to SEQ ID NO: 292
  Synthetic construct

SEQ ID NO: 315 - DNA, 79 bp, Artificial Sequence
  Synthetic construct
tggaaattcttccagaattgatactgactgtatgatgagagctgcaggtgtaatgaagaccttctttttgagatctggt

SEQ ID NO: 316 - DNA, 79 bp, Artificial Sequence
  Synthetic construct
tggaaattcttccagaattgatactgactgtatggtgagagctgcaggtgtaatgaagaccttctttttgagatctggt

SEQ ID NO: 317 - DNA, 78 bp, Artificial Sequence
  Synthetic construct
tggaaattcttccagaattgatactgactgtaaatgagagctgcaggtgtaatgaagaccttctttttgagatctggt

SEQ ID NO: 318 - DNA, 78 bp, Artificial Sequence
  Synthetic construct
tggaaattcttccagaattgatactgactgtatgtgagagctgcaggtgtaatgaagaccttctttttgagatctggt

SEQ ID NO: 319 - DNA, 74 bp, Artificial Sequence
  Synthetic construct
tggaaattcttccagaattgatactgaaaatgagagctgcaggtgtaatgaagaccttctttttgagatctggt

SEQ ID NO: 320 - DNA, 74 bp, Artificial Sequence
  Synthetic construct
tggaaattcttccagaattgatactgactgtatggactgcaggtgtaatgaagaccttctttttgagatctggt

SEQ ID NO: 321 - DNA, 74 bp, Artificial Sequence
  Synthetic construct
tggaaattcttccagaattgatactgactgtgagagctgcaggtgtaatgaagaccttctttttgagatctggt

SEQ ID NO: 322 - DNA, 73 bp, Artificial Sequence
  Synthetic construct
tggaaattcttccagaattgatactggtatgagagctgcaggtgtaatgaagaccttctttttgagatctggt

SEQ ID NO: 323 - DNA, 71 bp, Artificial Sequence
  Synthetic construct
tggaaattcttccagaattgatactgactgtagctgcaggtgtaatgaagaccttctttttgagatctggt

SEQ ID NO: 324 - DNA, 83 bp, Artificial Sequence; identical to SEQ ID NO: 292
  Synthetic construct

SEQ ID NO: 325 - DNA, 75 bp, Artificial Sequence
  Synthetic construct
tggaaattcttccagaattgatactgactgtatggaaactgcggtgtaatgaagaccttctttttgagatctggt

SEQ ID NO: 326 - DNA, 76 bp, Artificial Sequence
  Synthetic construct
tggaaattcttccagaattgatactgactgtatgagagctgcaggtgtaatgaagaccttctttttgagatctggt

SEQ ID NO: 327 - DNA, 74 bp, Artificial Sequence
  Synthetic construct
tggaaattcttccagaattaatactgactgtgagagctgcaggtgtaatgaagaccttctttttgagatctggt

SEQ ID NO: 328 - DNA, 73 bp, Artificial Sequence
  Synthetic construct
tggaaattcttccagaattgatactgactggagagctgcaggtgtaatgaagaccttctttttgagatctggt

SEQ ID NO: 329 - DNA, 72 bp, Artificial Sequence; identical to SEQ ID NO: 306
  Synthetic construct

SEQ ID NO: 330 - DNA, 68 bp, Artificial Sequence
  Synthetic construct
tggaaattcttccagaattgatactgactgctgcaggtgtaatgaagaccttctttttgagatctggt

SEQ ID NO: 331 - DNA, 65 bp, Artificial Sequence
  Synthetic construct
tggaaattcttccagaattgatactgactgtatgtgtaatgaagaccttctttttgagatctggt

SEQ ID NO: 332 - DNA, 39 bp, Artificial Sequence
  Synthetic construct
tggaaattcttccagaattgatactttttgagatctggt

SEQ ID NO: 333 - protein, 24 aa, Artificial Sequence
  Synthetic construct
RNNRNNRNNRNNNNYNNYNNYNNY

SEQ ID NO: 334 - protein, 24 aa, Artificial Sequence
  Synthetic construct
RNNRNNRNNRNNNNYNNYNNYNNY

SEQ ID NO: 335 - DNA, 20 bp, Artificial Sequence
  Synthetic construct
tccaaaaccatggtttacag

SEQ ID NO: 336 - DNA, 20 bp, Artificial Sequence
  Synthetic construct
tccaaaaccatggtttacag

SEQ ID NO: 337 - DNA, 20 bp, Artificial Sequence
  Synthetic construct
tccaaaaccatggtttacag

SEQ ID NO: 338 - DNA, 20 bp, Artificial Sequence
  Synthetic construct
tccaaaaccatggtttacag

SEQ ID NO: 339 - DNA, 20 bp, Artificial Sequence
  Synthetic construct
tccaaaaccatggtttacag

SEQ ID NO: 340 - DNA, 38 bp, Artificial Sequence
  Synthetic construct
  misc_feature (17)..(18): n is a, c, g, or t
  misc_feature (21)..(22): n is a, c, g, or t
ggaggcgtgtccaaaannatnntttacagcacgcctcc

SEQ ID NO: 341 - protein, 144 aa, Artificial Sequence
  Synthetic construct
MRLFGYARVSTSQQSLDIQVRALKDAGVKANRIFTDKASGSSCDRKGLDLLRMKVEEGDVILVKKLDRLGRDTADMIQLIKEFDAQGVSIRFIDDGISTDGEMGKMVVTILSAVAQAERQRILERTNEGRQEAMAKGVVFGRKR

SEQ ID NO: 342 - protein, 141 aa, Artificial Sequence
  Synthetic construct
MLIGYVRVSTNDQNTDLQRNALVCAGCEQIFEDKLSGTRTDRPGLKRALKRLQKGDTLVVWKLDRLGRSMKHLISLVGELRERGINFRSLTDSIDTSSPMGRFFFHVMGALAEMERELIIERTMAGLAAARNKGRIGGRPP

SEQ ID NO: 343 - DNA, 44 bp, Artificial Sequence
  Synthetic construct
  misc_feature (2)..(3): n is a, c, g, or t
  misc_feature (5)..(6): n is a, c, g, or t
  misc_feature (8)..(9): n is a, c, g, or t
  misc_feature (11)..(16): n is a, c, g, or t
  misc_feature (21)..(21): n is a, c, g, or t
  misc_feature (24)..(24): n is a, c, g, or t
  misc_feature (29)..(34): n is a, c, g, or t
  misc_feature (36)..(37): n is a, c, g, or t
  misc_feature (39)..(40): n is a, c, g, or t
  misc_feature (42)..(43): n is a, c, g, or t
rnnrnnrnnrnnnnnnaaabnwwnvtttnnnnnnynnynnynny

SEQ ID NO: 344 - DNA, 44 bp, Artificial Sequence
  Synthetic construct
gctgatgcagatacagaaaccaaggttttcttacttgctgctgc

SEQ ID NO: 345 - DNA, 44 bp, Artificial Sequence
  Synthetic construct
gtggatggagcagccaataggttcctttcctcccccttagcccc

SEQ ID NO: 346 - DNA, 44 bp, Artificial Sequence
  Synthetic construct
agggaagtcaatccagaaaccatcctttatcccttcctgtcctt

SEQ ID NO: 347 - DNA, 44 bp, Artificial Sequence
  Synthetic construct
ggaaatgtaaaagtagaaactaaagtttctgctttcattcttcc

SEQ ID NO: 348 - DNA, 44 bp, Artificial Sequence
  Synthetic construct
ggaagaaggatgagagaaactaacctttgtggaacccctgcagc

SEQ ID NO: 349 - DNA, 44 bp, Artificial Sequence
  Synthetic construct
aacggcagaagaagaaaaattatactttcttttccattgttttc

SEQ ID NO: 350 - DNA, 44 bp, Artificial Sequence
  Synthetic construct
gaggtaaatacttgataaatgttgcttttttcccccattaccct

SEQ ID NO: 351 - DNA, 44 bp, Artificial Sequence
  Synthetic construct
attgtggatggagtaaaaatgatcctttaatacatttctacatt

SEQ ID NO: 352 - DNA, 44 bp, Artificial Sequence
  Synthetic construct
ataggagaaaatttggaaagtataatttttcagactactctttt

SEQ ID NO: 353 - DNA, 43 bp, Artificial Sequence
  Synthetic construct
acagaagacattaagaaaacctaacttgacctcctatggttcc

SEQ ID NO: 354 - DNA, 44 bp, Artificial Sequence
  Synthetic construct
ggcaggacagctaactaatgaaaggtttggtgtgtgtctgtctt

SEQ ID NO: 355 - DNA, 44 bp, Artificial Sequence
  Synthetic construct
agggatgaggcctcataaagtaaagttttttgtttgtttgtttc

SEQ ID NO: 356 - DNA, 44 bp, Artificial Sequence
  Synthetic construct
acagtcaaagtatttgaaagttaacttttttcgtcagctcttcc

SEQ ID NO: 357 - DNA, 44 bp, Artificial Sequence
  Synthetic construct
gaaattgtggacaattaaattatcctttctgggccccttatttc

SEQ ID NO: 358 - DNA, 44 bp, Artificial Sequence
  Synthetic construct
gaaattggaaggaaaaaaattatcctttatggtgtaatacttat

SEQ ID NO: 359 - DNA, 44 bp, Artificial Sequence
  Synthetic construct
aaaacagctggctttgaaaggaaacttttaactactatcctgcc

SEQ ID NO: 360 - DNA, 44 bp, Artificial Sequence
  Synthetic construct
atagtaagtgctcaataaatgttcgtttatatcatcattgtggc

SEQ ID NO: 361 - DNA, 44 bp, Artificial Sequence
  Synthetic construct
aaagatggaacaaacaaaattaaggtttagtacattataattcc

SEQ ID NO: 362 - DNA, 43 bp, Artificial Sequence
  Synthetic construct
gcgggaggcgtgtccaaaccatggtttacagcacgcctcccgc

SEQ ID NO: 363 - DNA, 44 bp, Artificial Sequence
  Synthetic construct
gctgatgcagatcgagaaaccaaggttttcttacttgctgctgc

SEQ ID NO: 364 - DNA, 44 bp, Artificial Sequence; identical to SEQ ID NO: 345
  Synthetic construct

SEQ ID NO: 365 - DNA, 44 bp, Artificial Sequence; identical to SEQ ID NO: 346
  Synthetic construct

SEQ ID NO: 366 - DNA, 35 bp, Artificial Sequence
  Synthetic construct
agatacagaaaccgttttcttacttgctgctggcc

SEQ ID NO: 367 - DNA, 38 bp, Artificial Sequence
  Synthetic construct
tcagggaagtcatcctttatcccttcctgtccttagct

SEQ ID NO: 368 - DNA, 20 bp, Artificial Sequence
  Synthetic construct
  misc_feature (8)..(9): n is a, c, g, or t
  misc_feature (12)..(13): n is a, c, g, or t
tccasssnnatnnsssacag

SEQ ID NO: 369 - DNA, 20 bp, Artificial Sequence
  Synthetic construct
  misc_feature (1)..(4): n is a, c, g, or t
  misc_feature (8)..(9): n is a, c, g, or t
  misc_feature (12)..(13): n is a, c, g, or t
  misc_feature (17)..(20): n is a, c, g, or t
nnnnaaannatnntttnnnn